European Patent Specification EP 4 540 267 B1, published April 15, 2026. Title: CYCLIC PEPTIDES FOR TRAPPING INTERLEUKIN-1 BETA. Applicant: MERCK SHARP & DOHME LLC. The sequence listing filed with the application follows.

SEQUENCE LISTING (215 sequences)

SEQ ID NO: 1 - protein, 14 aa, synthetic construct
  SITE 1: note = (S)-3-(6-(4-acetylpiperazin-1-yl)pyridin-3-yl)-2-aminopropanoic acid
  SITE 3: note = l-phenylalanine-4-carboxylic acid
  SITE 5: note = (2S,4R)-4-aminopyrrolidine-2-carboxylic acid
  SITE 6: note = (2S,3S)-2-amino-3-(naphthalen-1-yl)butanoic acid
  SITE 8: note = d-N-methyl-Alanine
  SITE 10: note = l-Biphenylalanine-4-carboxylic acid
  SITE 11: note = 4-Pyridylalanine
  SITE 12: note = l-2,3-diaminopropionic acid
  SITE 13: note = d-Alanine
  SITE 14: note = (S)-2-amino-4-(5-cyanopyridin-3-yl)butanoic acid
XWXGXXDAGXXXAX

SEQ ID NO: 2 - protein, 14 aa, synthetic construct
  SITE 1: note = (S)-3-(6-(4-acetylpiperazin-1-yl)pyridin-3-yl)-2-aminopropanoic acid
  SITE 3: note = l-phenylalanine-4-carboxylic acid
  SITE 5: note = (2S,4R)-4-aminopyrrolidine-2-carboxylic acid
  SITE 6: note = (2S,3S)-2-amino-3-(naphthalen-1-yl)butanoic acid
  SITE 8: note = d-N-methyl-Alanine
  SITE 10: note = l-Biphenylalanine-4-carboxylic acid
  SITE 13: note = d-Alanine
  SITE 14: note = (S)-2-amino-4-(5-cyanopyridin-3-yl)butanoic acid
XWXGXXDAGXKLAX

SEQ ID NO: 3 - protein, 14 aa, synthetic construct
  SITE 1: note = (S)-3-(6-(4-acetylpiperazin-1-yl)pyridin-3-yl)-2-aminopropanoic acid
  SITE 3: note = l-phenylalanine-4-carboxylic acid
  SITE 5: note = (2S,4R)-4-aminopyrrolidine-2-carboxylic acid
  SITE 6: note = (2S,3S)-2-amino-3-(naphthalen-1-yl)butanoic acid
  SITE 8: note = d-N-methyl-Alanine
  SITE 10: note = l-Biphenylalanine-4-carboxylic acid
  SITE 13: note = d-Alanine
  SITE 14: note = l-homoTyrosine
XWXGXXDAGXKLAX

SEQ ID NO: 4 - protein, 14 aa, synthetic construct
  SITE 1: note = (S)-3-(6-(4-acetylpiperazin-1-yl)pyridin-3-yl)-2-aminopropanoic acid
  SITE 3: note = l-phenylalanine-4-carboxylic acid
  SITE 5: note = (2S,4R)-4-aminopyrrolidine-2-carboxylic acid
  SITE 6: note = (2S,3S)-2-amino-3-(naphthalen-1-yl)butanoic acid
  SITE 8: note = d-N-methyl-Alanine
  SITE 10: note = l-Biphenylalanine-4-carboxylic acid
  SITE 12: note = l-2,3-diaminopropionic acid
  SITE 13: note = d-Alanine
  SITE 14: note = (S)-2-amino-4-(5-cyanopyridin-3-yl)butanoic acid
XWXGXXDAGXWXAX

SEQ ID NO: 5 - protein, 14 aa, synthetic construct
  SITE 1: note = (S)-3-(6-(4-acetylpiperazin-1-yl)pyridin-3-yl)-2-aminopropanoic acid
  SITE 3: note = l-phenylalanine-4-carboxylic acid
  SITE 5: note = (2S,4R)-4-aminopyrrolidine-2-carboxylic acid
  SITE 6: note = (2S,3S)-2-amino-3-(naphthalen-1-yl)butanoic acid
  SITE 8: note = d-N-methyl-Alanine
  SITE 10: note = l-Biphenylalanine-4-carboxylic acid
  SITE 12: note = l-2,3-diaminopropionic acid
  SITE 13: note = d-Alanine
  SITE 14: note = l-homoTyrosine
XWXGXXDAGXWXAX

SEQ ID NO: 6 - protein, 14 aa, synthetic construct
  SITE 1: note = (S)-3-(6-(4-acetylpiperazin-1-yl)pyridin-3-yl)-2-aminopropanoic acid
  SITE 3: note = l-phenylalanine-4-carboxylic acid
  SITE 5: note = (2S,4R)-4-aminopyrrolidine-2-carboxylic acid
  SITE 6: note = (2S,3S)-2-amino-3-(4-fluoro-1H-indol-3-yl)butanoic acid
  SITE 8: note = d-N-methyl-Alanine
  SITE 10: note = l-Biphenylalanine-4-carboxylic acid
  SITE 13: note = d-Alanine
  SITE 14: note = l-homoTyrosine
XWXGXXDAGXKLAX

SEQ ID NO: 7 - protein, 14 aa, synthetic construct
  SITE 1: note = (S)-3-(6-(4-acetylpiperazin-1-yl)pyridin-3-yl)-2-aminopropanoic acid
  SITE 3: note = l-phenylalanine-4-carboxylic acid
  SITE 5: note = (2S,4R)-4-aminopyrrolidine-2-carboxylic acid
  SITE 6: note = (2S,3S)-2-amino-3-(4-fluoro-1H-indol-3-yl)butanoic acid
  SITE 8: note = d-N-methyl-Alanine
  SITE 10: note = l-Biphenylalanine-4-carboxylic acid
  SITE 13: note = d-2,4-diaminobutyric acid
  SITE 14: note = l-homoTyrosine
XWXGXXDAGXKLXX

SEQ ID NO: 8 - protein, 14 aa, synthetic construct
  SITE 1: note = (S)-3-(6-(4-acetylpiperazin-1-yl)pyridin-3-yl)-2-aminopropanoic acid
  SITE 3: note = l-phenylalanine-4-carboxylic acid
  SITE 5: note = (2S,4R)-4-aminopyrrolidine-2-carboxylic acid
  SITE 6: note = (2S,3S)-2-amino-3-(4-fluoro-1H-indol-3-yl)butanoic acid
  SITE 8: note = d-N-methyl-Alanine
  SITE 10: note = l-Biphenylalanine-4-carboxylic acid
  SITE 13: note = d-2,4-diaminobutyric acid
  SITE 14: note = l-homoTyrosine
XWXGXXDAGXWGXX

SEQ ID NO: 9 - protein, 14 aa, synthetic construct
  SITE 1: note = (S)-3-(6-(2-acetamidoethoxy)pyridin-3-yl)-2-aminopropanoic acid
  SITE 3: note = l-phenylalanine-4-carboxylic acid
  SITE 5: note = (2S,4R)-4-aminopyrrolidine-2-carboxylic acid
  SITE 6: note = (2S,3S)-2-amino-3-(4-fluoro-1H-indol-3-yl)butanoic acid
  SITE 8: note = d-N-methyl-Alanine
  SITE 10: note = l-Biphenylalanine-4-carboxylic acid
  SITE 13: note = d-Alanine
  SITE 14: note = l-homoTyrosine
XWXGXXDAGXKLAX

SEQ ID NO: 10 - protein, 14 aa, synthetic construct
  SITE 1: note = (S)-4-(5-(2-amino-2-carboxyethyl)pyridin-2-yl)benzoic acid
  SITE 3: note = l-phenylalanine-4-carboxylic acid
  SITE 5: note = (2S,4R)-4-aminopyrrolidine-2-carboxylic acid
  SITE 6: note = (2S,3S)-2-amino-3-(naphthalen-1-yl)butanoic acid
  SITE 8: note = d-N-methyl-Alanine
  SITE 10: note = (S)-4-(5-(2-amino-2-carboxyethyl)pyridin-2-yl)benzoic acid
  SITE 12: note = l-2,3-diaminopropionic acid
  SITE 13: note = d-Alanine
  SITE 14: note = l-homoTyrosine
XWXGXXDAGXWXAX

SEQ ID NO: 11 - protein, 14 aa, synthetic construct
  SITE 1: note = (S)-4-(5-(2-amino-2-carboxyethyl)pyridin-2-yl)benzoic acid
  SITE 3: note = l-phenylalanine-4-carboxylic acid
  SITE 5: note = (2S,4R)-4-aminopyrrolidine-2-carboxylic acid
  SITE 6: note = (2S,3S)-2-amino-3-(naphthalen-1-yl)butanoic acid
  SITE 8: note = d-N-methyl-Alanine
  SITE 10: note = l-Biphenylalanine-4-carboxylic acid
  SITE 12: note = l-2,3-diaminopropionic acid
  SITE 13: note = d-Alanine
  SITE 14: note = l-homoTyrosine
XWXGXXDAGXWXAX

SEQ ID NO: 12 - protein, 14 aa, synthetic construct
  SITE 1: note = l-Biphenylalanine-4-carboxylic acid
  SITE 3: note = l-phenylalanine-4-carboxylic acid
  SITE 5: note = (2S,4R)-4-aminopyrrolidine-2-carboxylic acid
  SITE 6: note = (2S,3S)-2-amino-3-(naphthalen-1-yl)butanoic acid
  SITE 8: note = d-N-methyl-Alanine
  SITE 10: note = (S)-4-(5-(2-amino-2-carboxyethyl)pyridin-2-yl)benzoic acid
  SITE 12: note = l-2,3-diaminopropionic acid
  SITE 13: note = d-Alanine
  SITE 14: note = l-homoTyrosine
XWXGXXDAGXWXAX

SEQ ID NO: 13 - protein, 14 aa, synthetic construct
  SITE 1: note = l-Biphenylalanine-4-carboxylic acid
  SITE 3: note = l-phenylalanine-4-carboxylic acid
  SITE 5: note = (2S,4R)-4-aminopyrrolidine-2-carboxylic acid
  SITE 6: note = (2S,3S)-2-amino-3-(naphthalen-1-yl)butanoic acid
  SITE 8: note = d-N-methyl-Alanine
  SITE 10: note = l-Biphenylalanine-4-carboxylic acid
  SITE 11: note = (S)-2-amino-3-(1H-indazol-1-yl)propanoic acid
  SITE 12: note = l-2,3-diaminopropionic acid
  SITE 13: note = d-Alanine
  SITE 14: note = l-homoTyrosine
XWXGXXDAGXXXAX

SEQ ID NO: 14 - protein, 14 aa, synthetic construct
  SITE 1: note = l-Biphenylalanine-4-carboxylic acid
  SITE 3: note = l-phenylalanine-4-carboxylic acid
  SITE 5: note = (2S,4R)-4-aminopyrrolidine-2-carboxylic acid
  SITE 6: note = (2S,3S)-2-amino-3-(naphthalen-1-yl)butanoic acid
  SITE 8: note = d-N-methyl-Alanine
  SITE 10: note = l-Biphenylalanine-4-carboxylic acid
  SITE 11: note = (S)-2-amino-3-(indolin-1-yl)propanoic acid
  SITE 12: note = l-2,3-diaminopropionic acid
  SITE 13: note = d-Alanine
  SITE 14: note = l-homoTyrosine
XWXGXXDAGXXXAX

SEQ ID NO: 15 - protein, 14 aa, synthetic construct
  SITE 1: note = l-Biphenylalanine-4-carboxylic acid
  SITE 3: note = l-phenylalanine-4-carboxylic acid
  SITE 5: note = (2S,4R)-4-aminopyrrolidine-2-carboxylic acid
  SITE 6: note = (2S,3S)-2-amino-3-(naphthalen-1-yl)butanoic acid
  SITE 8: note = d-N-methyl-Alanine
  SITE 10: note = l-Biphenylalanine-4-carboxylic acid
  SITE 11: note = 3-(1-Naphthyl)-l-alanine
  SITE 12: note = l-2,4-diaminobutyric acid
  SITE 13: note = Aminoisobutyric acid
XWXGXXDAGXXXXG

SEQ ID NO: 16 - protein, 14 aa, synthetic construct
  SITE 1: note = l-Biphenylalanine-4-carboxylic acid
  SITE 3: note = l-phenylalanine-4-carboxylic acid
  SITE 5: note = (2S,4R)-4-aminopyrrolidine-2-carboxylic acid
  SITE 6: note = (2S,3S)-2-amino-3-(naphthalen-1-yl)butanoic acid
  SITE 8: note = d-N-methyl-Alanine
  SITE 10: note = l-Biphenylalanine-4-carboxylic acid
  SITE 11: note = 3-(1-Naphthyl)-l-alanine
  SITE 12: note = l-2,4-diaminobutyric acid
  SITE 13: note = Aminoisobutyric acid
  SITE 14: note = l-homoTyrosine
XWXGXXDAGXXXXX

SEQ ID NO: 17 - protein, 14 aa, synthetic construct
  SITE 1: note = l-Biphenylalanine-4-carboxylic acid
  SITE 3: note = l-phenylalanine-4-carboxylic acid
  SITE 5: note = (2S,4R)-4-aminopyrrolidine-2-carboxylic acid
  SITE 6: note = (2S,3S)-2-amino-3-(naphthalen-1-yl)butanoic acid
  SITE 8: note = d-N-methyl-Alanine
  SITE 10: note = l-Biphenylalanine-4-carboxylic acid
  SITE 11: note = 3-(1-Naphthyl)-l-alanine
  SITE 12: note = l-2,3-diaminopropionic acid
  SITE 13: note = Aminoisobutyric acid
XWXGXXDAGXXXXG

SEQ ID NO: 18 - protein, 14 aa, synthetic construct
  SITE 1: note = l-Biphenylalanine-4-carboxylic acid
  SITE 3: note = l-phenylalanine-4-carboxylic acid
  SITE 5: note = (2S,4R)-4-aminopyrrolidine-2-carboxylic acid
  SITE 6: note = (2S,3S)-2-amino-3-(naphthalen-1-yl)butanoic acid
  SITE 8: note = d-N-methyl-Alanine
  SITE 10: note = l-Biphenylalanine-4-carboxylic acid
  SITE 11: note = 3-(1-Naphthyl)-l-alanine
  SITE 12: note = l-2,3-diaminopropionic acid
  SITE 13: note = Aminoisobutyric acid
  SITE 14: note = (S)-2-amino-4-(5-cyanopyridin-3-yl)butanoic acid
XWXGXXDAGXXXXX

SEQ ID NO: 19 - protein, 14 aa, synthetic construct
  SITE 1: note = l-Biphenylalanine-4-carboxylic acid
  SITE 3: note = l-phenylalanine-4-carboxylic acid
  SITE 5: note = (2S,4R)-4-aminopyrrolidine-2-carboxylic acid
  SITE 6: note = (2S,3S)-2-amino-3-(naphthalen-1-yl)butanoic acid
  SITE 8: note = d-N-methyl-Alanine
  SITE 10: note = l-Biphenylalanine-4-carboxylic acid
  SITE 11: note = 3-(1-Naphthyl)-l-alanine
  SITE 13: note = Aminoisobutyric acid
XWXGXXDAGXXLXG

SEQ ID NO: 20 - protein, 14 aa, synthetic construct
  SITE 1: note = l-Biphenylalanine-4-carboxylic acid
  SITE 3: note = l-phenylalanine-4-carboxylic acid
  SITE 5: note = (2S,4R)-4-aminopyrrolidine-2-carboxylic acid
  SITE 6: note = (2S,3S)-2-amino-3-(naphthalen-1-yl)butanoic acid
  SITE 8: note = d-N-methyl-Alanine
  SITE 10: note = l-Biphenylalanine-4-carboxylic acid
  SITE 11: note = 3-(1-Naphthyl)-l-alanine
  SITE 12: note = l-Ornithine
  SITE 13: note = Aminoisobutyric acid
XWXGXXDAGXXXXG

SEQ ID NO: 21 - protein, 14 aa, synthetic construct
  SITE 1: note = l-Biphenylalanine-4-carboxylic acid
  SITE 3: note = l-phenylalanine-4-carboxylic acid
  SITE 5: note = (2S,4R)-4-aminopyrrolidine-2-carboxylic acid
  SITE 6: note = (2S,3S)-2-amino-3-(naphthalen-1-yl)butanoic acid
  SITE 8: note = d-N-methyl-Alanine
  SITE 10: note = l-Biphenylalanine-4-carboxylic acid
  SITE 11: note = 4-Pyridylalanine
  SITE 12: note = l-2,3-diaminopropionic acid
  SITE 13: note = d-Alanine
  SITE 14: note = (S)-2-amino-4-(5-cyanopyridin-3-yl)butanoic acid
XWXGXXDAGXXXAX

SEQ ID NO: 22 - protein, 14 aa, synthetic construct
  SITE 1: note = l-Biphenylalanine-4-carboxylic acid
  SITE 3: note = l-phenylalanine-4-carboxylic acid
  SITE 5: note = (2S,4R)-4-aminopyrrolidine-2-carboxylic acid
  SITE 6: note = (2S,3S)-2-amino-3-(naphthalen-1-yl)butanoic acid
  SITE 8: note = d-N-methyl-Alanine
  SITE 10: note = l-Biphenylalanine-4-carboxylic acid
  SITE 11: note = 4-Pyridylalanine
  SITE 12: note = l-2,3-diaminopropionic acid
  SITE 13: note = d-Alanine
  SITE 14: note = l-homoTyrosine
XWXGXXDAGXXXAX

SEQ ID NO: 23 - protein, 14 aa, synthetic construct
  SITE 1: note = l-Biphenylalanine-4-carboxylic acid
  SITE 3: note = l-phenylalanine-4-carboxylic acid
  SITE 5: note = (2S,4R)-4-aminopyrrolidine-2-carboxylic acid
  SITE 6: note = (2S,3S)-2-amino-3-(naphthalen-1-yl)butanoic acid
  SITE 8: note = d-N-methyl-Alanine
  SITE 10: note = l-Biphenylalanine-4-carboxylic acid
  SITE 11: note = (S)-2-amino-3-(tetrahydro-2H-pyran-4-yl)propanoic acid
  SITE 12: note = l-2,3-diaminopropionic acid
  SITE 13: note = d-Alanine
  SITE 14: note = (S)-2-amino-4-(5-cyanopyridin-3-yl)butanoic acid
XWXGXXDAGXXXAX

SEQ ID NO: 24 - protein, 14 aa, synthetic construct
  SITE 1: note = l-Biphenylalanine-4-carboxylic acid
  SITE 3: note = l-phenylalanine-4-carboxylic acid
  SITE 5: note = (2S,4R)-4-aminopyrrolidine-2-carboxylic acid
  SITE 6: note = (2S,3S)-2-amino-3-(naphthalen-1-yl)butanoic acid
  SITE 8: note = d-N-methyl-Alanine
  SITE 10: note = l-Biphenylalanine-4-carboxylic acid
  SITE 11: note = (S)-2-amino-3-(tetrahydro-2H-pyran-4-yl)propanoic acid
  SITE 12: note = l-2,3-diaminopropionic acid
  SITE 13: note = d-Alanine
  SITE 14: note = l-homoTyrosine
XWXGXXDAGXXXAX

SEQ ID NO: 25 - protein, 14 aa, synthetic construct
  SITE 1: note = l-Biphenylalanine-4-carboxylic acid
  SITE 3: note = l-phenylalanine-4-carboxylic acid
  SITE 5: note = (2S,4R)-4-aminopyrrolidine-2-carboxylic acid
  SITE 6: note = (2S,3S)-2-amino-3-(naphthalen-1-yl)butanoic acid
  SITE 8: note = d-N-methyl-Alanine
  SITE 10: note = l-Biphenylalanine-4-carboxylic acid
  SITE 13: note = d-Alanine
  SITE 14: note = l-homoTyrosine
XWXGXXDAGXKLAX

SEQ ID NO: 26 - protein, 14 aa, synthetic construct
  SITE 1: note = l-Biphenylalanine-4-carboxylic acid
  SITE 3: note = l-phenylalanine-4-carboxylic acid
  SITE 5: note = (2S,4R)-4-aminopyrrolidine-2-carboxylic acid
  SITE 6: note = (2S,3S)-2-amino-3-(naphthalen-1-yl)butanoic acid
  SITE 8: note = d-N-methyl-Alanine
  SITE 10: note = l-Biphenylalanine-4-carboxylic acid
  SITE 13: note = d-Serine
  SITE 14: note = l-homoTyrosine
XWXGXXDAGXKLSX

SEQ ID NO: 27 - protein, 14 aa, synthetic construct
  SITE 1: note = l-Biphenylalanine-4-carboxylic acid
  SITE 3: note = l-phenylalanine-4-carboxylic acid
  SITE 5: note = (2S,4R)-4-aminopyrrolidine-2-carboxylic acid
  SITE 6: note = (2S,3S)-2-amino-3-(naphthalen-1-yl)butanoic acid
  SITE 8: note = d-N-methyl-Alanine
  SITE 10: note = l-Biphenylalanine-4-carboxylic acid
  SITE 11: note = (S)-2-amino-3-(pyrimidin-5-yl)propanoic acid
  SITE 12: note = l-2,3-diaminopropionic acid
  SITE 13: note = d-Alanine
  SITE 14: note = (S)-2-amino-4-(5-cyanopyridin-3-yl)butanoic acid
XWXGXXDAGXXXAX

SEQ ID NO: 28 - protein, 14 aa, synthetic construct
  SITE 1: note = l-Biphenylalanine-4-carboxylic acid
  SITE 3: note = l-phenylalanine-4-carboxylic acid
  SITE 5: note = (2S,4R)-4-aminopyrrolidine-2-carboxylic acid
  SITE 6: note = (2S,3S)-2-amino-3-(naphthalen-1-yl)butanoic acid
  SITE 8: note = d-N-methyl-Alanine
  SITE 10: note = l-Biphenylalanine-4-carboxylic acid
  SITE 11: note = (S)-2-amino-3-(pyrimidin-5-yl)propanoic acid
  SITE 12: note = l-2,3-diaminopropionic acid
  SITE 13: note = d-Alanine
  SITE 14: note = l-homoTyrosine
XWXGXXDAGXXXAX

SEQ ID NO: 29 - protein, 14 aa, synthetic construct
  SITE 1: note = l-Biphenylalanine-4-carboxylic acid
  SITE 3: note = l-phenylalanine-4-carboxylic acid
  SITE 5: note = (2S,4R)-4-aminopyrrolidine-2-carboxylic acid
  SITE 6: note = (2S,3S)-2-amino-3-(naphthalen-1-yl)butanoic acid
  SITE 8: note = d-N-methyl-Alanine
  SITE 10: note = l-Biphenylalanine-4-carboxylic acid
  SITE 11: note = (S)-2-amino-3-(1H-pyrrolo[2,3-b]pyridin-3-yl)propanoic acid
  SITE 12: note = l-2,3-diaminopropionic acid
  SITE 13: note = d-Alanine
  SITE 14: note = l-homoTyrosine
XWXGXXDAGXXXAX

SEQ ID NO: 30 - protein, 14 aa, synthetic construct
  SITE 1: note = l-Biphenylalanine-4-carboxylic acid
  SITE 3: note = l-phenylalanine-4-carboxylic acid
  SITE 5: note = (2S,4R)-4-aminopyrrolidine-2-carboxylic acid
  SITE 6: note = (2S,3S)-2-amino-3-(naphthalen-1-yl)butanoic acid
  SITE 8: note = d-N-methyl-Alanine
  SITE 10: note = l-Biphenylalanine-4-carboxylic acid
  SITE 12: note = l-2,3-diaminopropionic acid
  SITE 13: note = d-Alanine
  SITE 14: note = (S)-2-amino-4-(5-cyanopyridin-3-yl)butanoic acid
XWXGXXDAGXWXAX

SEQ ID NO: 31 - protein, 14 aa, synthetic construct
  SITE 1: note = l-Biphenylalanine-4-carboxylic acid
  SITE 3: note = l-phenylalanine-4-carboxylic acid
  SITE 5: note = (2S,4R)-4-aminopyrrolidine-2-carboxylic acid
  SITE 6: note = (2S,3S)-2-amino-3-(naphthalen-1-yl)butanoic acid
  SITE 8: note = d-N-methyl-Alanine
  SITE 10: note = l-Biphenylalanine-4-carboxylic acid
  SITE 12: note = l-2,3-diaminopropionic acid
  SITE 13: note = d-Alanine
  SITE 14: note = l-homoTyrosine
XWXGXXDAGXWXAX

SEQ ID NO: 32 - protein, 14 aa, synthetic construct
  SITE 1: note = l-Biphenylalanine-4-carboxylic acid
  SITE 3: note = l-phenylalanine-4-carboxylic acid
  SITE 5: note = (2S,4R)-4-aminopyrrolidine-2-carboxylic acid
  SITE 6: note = (2S,3S)-2-amino-3-(naphthalen-1-yl)butanoic acid
  SITE 8: note = d-N-methyl-Alanine
  SITE 10: note = l-Biphenylalanine-4-carboxylic acid
  SITE 13: note = d-2,4-diaminobutyric acid
  SITE 14: note = l-homoTyrosine
XWXGXXDAGXWGXX

SEQ ID NO: 33 - protein, 14 aa, synthetic construct
  SITE 1: note = l-Biphenylalanine-4-carboxylic acid
  SITE 3: note = l-phenylalanine-4-carboxylic acid
  SITE 5: note = (2S,4R)-4-aminopyrrolidine-2-carboxylic acid
  SITE 6: note = (2S,3S)-2-amino-3-(4-chloro-1H-indol-3-yl)butanoic acid
  SITE 8: note = d-N-methyl-Alanine
  SITE 10: note = l-Biphenylalanine-4-carboxylic acid
  SITE 11: note = 3-(1-Naphthyl)-l-alanine
  SITE 13: note = Aminoisobutyric acid
XWXGXXAAGXXLXG

SEQ ID NO: 34 - protein, 14 aa, synthetic construct
  SITE 1: note = l-Biphenylalanine-4-carboxylic acid
  SITE 3: note = l-phenylalanine-4-carboxylic acid
  SITE 5: note = (2S,4R)-4-aminopyrrolidine-2-carboxylic acid
  SITE 6: note = (2S,3S)-2-amino-3-(4-chloro-1H-indol-3-yl)butanoic acid
  SITE 8: note = d-N-methyl-Alanine
  SITE 10: note = l-Biphenylalanine-4-carboxylic acid
  SITE 11: note = 3-(1-Naphthyl)-l-alanine
  SITE 12: note = l-2,3-diaminopropionic acid
  SITE 13: note = Aminoisobutyric acid
  SITE 14: note = (S)-2-amino-4-(5-cyanopyridin-3-yl)butanoic acid
XWXGXXDAGXXXXX

SEQ ID NO: 35 - protein, 14 aa, synthetic construct
  SITE 1: note = l-Biphenylalanine-4-carboxylic acid
  SITE 3: note = l-phenylalanine-4-carboxylic acid
  SITE 5: note = (2S,4R)-4-aminopyrrolidine-2-carboxylic acid
  SITE 6: note = (2S,3S)-2-amino-3-(4-chloro-1H-indol-3-yl)butanoic acid
  SITE 8: note = d-N-methyl-Alanine
  SITE 10: note = l-Biphenylalanine-4-carboxylic acid
  SITE 11: note = 3-(1-Naphthyl)-l-alanine
  SITE 13: note = Aminoisobutyric acid
XWXGXXDAGXXLXG

SEQ ID NO: 36 - protein, 14 aa, synthetic construct
  SITE 1: note = l-Biphenylalanine-4-carboxylic acid
  SITE 3: note = l-phenylalanine-4-carboxylic acid
  SITE 5: note = (2S,4R)-4-aminopyrrolidine-2-carboxylic acid
  SITE 6: note = (2S,3S)-2-amino-3-(4-chloro-1H-indol-3-yl)butanoic acid
  SITE 8: note = d-N-methyl-Alanine
  SITE 10: note = l-Biphenylalanine-4-carboxylic acid
  SITE 11: note = 3-(1-Naphthyl)-l-alanine
  SITE 13: note = Aminoisobutyric acid
  SITE 14: note = l-homoTyrosine
XWXGXXDAGXXLXX

SEQ ID NO: 37 - protein, 14 aa, synthetic construct
  SITE 1: note = l-Biphenylalanine-4-carboxylic acid
  SITE 3: note = l-phenylalanine-4-carboxylic acid
  SITE 5: note = (2S,4R)-4-aminopyrrolidine-2-carboxylic acid
  SITE 6: note = (2S,3S)-2-amino-3-(4-chloro-1H-indol-3-yl)butanoic acid
  SITE 8: note = d-N-methyl-Alanine
  SITE 10: note = l-Biphenylalanine-4-carboxylic acid
  SITE 11: note = 3-(1-Naphthyl)-l-alanine
  SITE 12: note = l-Ornithine
  SITE 13: note = Aminoisobutyric acid
XWXGXXDAGXXXXG

SEQ ID NO: 38 - protein, 14 aa, synthetic construct
  SITE 1: note = l-Biphenylalanine-4-carboxylic acid
  SITE 3: note = l-phenylalanine-4-carboxylic acid
  SITE 5: note = (2S,4R)-4-aminopyrrolidine-2-carboxylic acid
  SITE 6: note = (2S,3S)-2-amino-3-(4-chloro-1H-indol-3-yl)butanoic acid
  SITE 8: note = d-N-methyl-Alanine
  SITE 10: note = l-Biphenylalanine-4-carboxylic acid
  SITE 11: note = 3-Pyridylalanine
  SITE 13: note = d-Alanine
  SITE 14: note = l-homoTyrosine
XWXGXXDAGXXSAX

SEQ ID NO: 39 - protein, 14 aa, synthetic construct
  SITE 1: note = l-Biphenylalanine-4-carboxylic acid
  SITE 3: note = l-phenylalanine-4-carboxylic acid
  SITE 5: note = (2S,4R)-4-aminopyrrolidine-2-carboxylic acid
  SITE 6: note = (2S,3S)-2-amino-3-(4-chloro-1H-indol-3-yl)butanoic acid
  SITE 8: note = d-N-methyl-Alanine
  SITE 10: note = l-Biphenylalanine-4-carboxylic acid
  SITE 11: note = 4-Pyridylalanine
  SITE 13: note = d-Alanine
  SITE 14: note = l-homoTyrosine
XWXGXXDAGXXSAX

SEQ ID NO: 40 - protein, 14 aa, synthetic construct
  SITE 1: note = l-Biphenylalanine-4-carboxylic acid
  SITE 3: note = l-phenylalanine-4-carboxylic acid
  SITE 5: note = (2S,4R)-4-aminopyrrolidine-2-carboxylic acid
  SITE 6: note = (2S,3S)-2-amino-3-(4-chloro-1H-indol-3-yl)butanoic acid
  SITE 8: note = d-N-methyl-Alanine
  SITE 10: note = l-Biphenylalanine-4-carboxylic acid
  SITE 11: note = (S)-2-amino-3-(piperidin-4-yl)propanoic acid
  SITE 13: note = d-Alanine
  SITE 14: note = l-homoTyrosine
XWXGXXDAGXXSAX

SEQ ID NO: 41 - protein, 14 aa, synthetic construct
  SITE 1: note = l-Biphenylalanine-4-carboxylic acid
  SITE 3: note = l-phenylalanine-4-carboxylic acid
  SITE 5: note = (2S,4R)-4-aminopyrrolidine-2-carboxylic acid
  SITE 6: note = (2S,3S)-2-amino-3-(4-chloro-1H-indol-3-yl)butanoic acid
  SITE 8: note = d-N-methyl-Alanine
  SITE 10: note = l-Biphenylalanine-4-carboxylic acid
  SITE 11: note = l-2,3-diaminopropionic acid
  SITE 13: note = d-Alanine
  SITE 14: note = l-homoTyrosine
XWXGXXDAGXXSAX

SEQ ID NO: 42 - protein, 14 aa, synthetic construct
  SITE 1: note = l-Biphenylalanine-4-carboxylic acid
  SITE 3: note = l-phenylalanine-4-carboxylic acid
  SITE 5: note = (2S,4R)-4-aminopyrrolidine-2-carboxylic acid
  SITE 6: note = (2S,3S)-2-amino-3-(4-chloro-1H-indol-3-yl)butanoic acid
  SITE 8: note = d-N-methyl-Alanine
  SITE 10: note = l-Biphenylalanine-4-carboxylic acid
  SITE 13: note = d-Alanine
  SITE 14: note = l-homoTyrosine
XWXGXXDAGXKLAX

SEQ ID NO: 43 - protein, 14 aa, synthetic construct
  SITE 1: note = l-Biphenylalanine-4-carboxylic acid
  SITE 3: note = l-phenylalanine-4-carboxylic acid
  SITE 5: note = (2S,4R)-4-aminopyrrolidine-2-carboxylic acid
  SITE 6: note = (2S,3S)-2-amino-3-(4-chloro-1H-indol-3-yl)butanoic acid
  SITE 8: note = d-N-methyl-Alanine
  SITE 10: note = l-Biphenylalanine-4-carboxylic acid
  SITE 13: note = d-2,4-diaminobutyric acid
  SITE 14: note = l-homoTyrosine
XWXGXXDAGXKLXX

SEQ ID NO: 44 - protein, 14 aa, synthetic construct
  SITE 1: note = l-Biphenylalanine-4-carboxylic acid
  SITE 3: note = l-phenylalanine-4-carboxylic acid
  SITE 5: note = (2S,4R)-4-aminopyrrolidine-2-carboxylic acid
  SITE 6: note = (2S,3S)-2-amino-3-(4-chloro-1H-indol-3-yl)butanoic acid
  SITE 8: note = d-N-methyl-Alanine
  SITE 10: note = l-Biphenylalanine-4-carboxylic acid
  SITE 13: note = d-Serine
  SITE 14: note = l-homoTyrosine
XWXGXXDAGXKLSX

SEQ ID NO: 45 - protein, 14 aa, synthetic construct
  SITE 1: note = l-Biphenylalanine-4-carboxylic acid
  SITE 3: note = l-phenylalanine-4-carboxylic acid
  SITE 5: note = (2S,4R)-4-aminopyrrolidine-2-carboxylic acid
  SITE 6: note = (2S,3S)-2-amino-3-(4-chloro-1H-indol-3-yl)butanoic acid
  SITE 8: note = d-N-methyl-Alanine
  SITE 10: note = l-Biphenylalanine-4-carboxylic acid
  SITE 13: note = d-Alanine
  SITE 14: note = l-homoTyrosine
XWXGXXDAGXKSAX

SEQ ID NO: 46 - protein, 14 aa, synthetic construct
  SITE 1: note = l-Biphenylalanine-4-carboxylic acid
  SITE 3: note = l-phenylalanine-4-carboxylic acid
  SITE 5: note = (2S,4R)-4-aminopyrrolidine-2-carboxylic acid
  SITE 6: note = (2S,3S)-2-amino-3-(4-chloro-1H-indol-3-yl)butanoic acid
  SITE 8: note = d-N-methyl-Alanine
  SITE 10: note = l-Biphenylalanine-4-carboxylic acid
  SITE 13: note = d-2,4-diaminobutyric acid
  SITE 14: note = l-homoTyrosine
XWXGXXDAGXKSXX

SEQ ID NO: 47 - protein, 14 aa, synthetic construct
  SITE 1: note = l-Biphenylalanine-4-carboxylic acid
  SITE 3: note = l-phenylalanine-4-carboxylic acid
  SITE 5: note = (2S,4R)-4-aminopyrrolidine-2-carboxylic acid
  SITE 6: note = (2S,3S)-2-amino-3-(4-chloro-1H-indol-3-yl)butanoic acid
  SITE 8: note = d-N-methyl-Alanine
  SITE 10: note = l-Biphenylalanine-4-carboxylic acid
  SITE 13: note = d-Serine
  SITE 14: note = l-homoTyrosine
XWXGXXDAGXKSSX

SEQ ID NO: 48 - protein, 14 aa, synthetic construct
  SITE 1: note = l-Biphenylalanine-4-carboxylic acid
  SITE 3: note = l-phenylalanine-4-carboxylic acid
  SITE 5: note = (2S,4R)-4-aminopyrrolidine-2-carboxylic acid
  SITE 6: note = (2S,3S)-2-amino-3-(4-chloro-1H-indol-3-yl)butanoic acid
  SITE 8: note = d-N-methyl-Alanine
  SITE 10: note = l-Biphenylalanine-4-carboxylic acid
  SITE 11: note = (S)-2-amino-3-(3-(aminomethyl)phenyl)propanoic acid
  SITE 13: note = d-Alanine
  SITE 14: note = l-homoTyrosine
XWXGXXDAGXXSAX

SEQ ID NO: 49 - protein, 14 aa, synthetic construct
  SITE 1: note = l-Biphenylalanine-4-carboxylic acid
  SITE 3: note = l-phenylalanine-4-carboxylic acid
  SITE 5: note = (2S,4R)-4-aminopyrrolidine-2-carboxylic acid
  SITE 6: note = (2S,3S)-2-amino-3-(4-chloro-1H-indol-3-yl)butanoic acid
  SITE 8: note = d-N-methyl-Alanine
  SITE 10: note = l-Biphenylalanine-4-carboxylic acid
  SITE 11: note = l-Ornithine
  SITE 13: note = d-Alanine
  SITE 14: note = l-homoTyrosine
XWXGXXDAGXXSAX

SEQ ID NO: 50 - protein, 14 aa, synthetic construct
  SITE 1: note = l-Biphenylalanine-4-carboxylic acid
  SITE 3: note = l-phenylalanine-4-carboxylic acid
  SITE 5: note = (2S,4R)-4-aminopyrrolidine-2-carboxylic acid
  SITE 6: note = (2S,3S)-2-amino-3-(4-chloro-1H-indol-3-yl)butanoic acid
  SITE 8: note = d-N-methyl-Alanine
  SITE 10: note = l-Biphenylalanine-4-carboxylic acid
  SITE 11: note = (S)-2-amino-3-(3-aminophenyl)propanoic acid
  SITE 13: note = d-Alanine
  SITE 14: note = l-homoTyrosine
XWXGXXDAGXXSAX

SEQ ID NO: 51 - protein, 14 aa, synthetic construct
  SITE 1: note = l-Biphenylalanine-4-carboxylic acid
  SITE 3: note = l-phenylalanine-4-carboxylic acid
  SITE 5: note = (2S,4R)-4-aminopyrrolidine-2-carboxylic acid
  SITE 6: note = (2S,3S)-2-amino-3-(4-chloro-1H-indol-3-yl)butanoic acid
  SITE 8: note = d-N-methyl-Alanine
  SITE 10: note = l-Biphenylalanine-4-carboxylic acid
  SITE 11: note = (S)-2-amino-3-[4-(aminomethyl)phenyl]propanoic acid
  SITE 13: note = d-Alanine
  SITE 14: note = l-homoTyrosine
XWXGXXDAGXXSAX

SEQ ID NO: 52 - protein, 14 aa, synthetic construct
  SITE 1: note = l-Biphenylalanine-4-carboxylic acid
  SITE 3: note = l-phenylalanine-4-carboxylic acid
  SITE 5: note = (2S,4R)-4-aminopyrrolidine-2-carboxylic acid
  SITE 6: note = (2S,3S)-2-amino-3-(4-chloro-1H-indol-3-yl)butanoic acid
  SITE 8: note = d-N-methyl-Alanine
  SITE 10: note = l-Biphenylalanine-4-carboxylic acid
  SITE 11: note = (S)-2-amino-3-(4-aminophenyl)propanoic acid
  SITE 13: note = d-Alanine
  SITE 14: note = l-homoTyrosine
XWXGXXDAGXXSAX

SEQ ID NO: 53 - protein, 14 aa, synthetic construct
  SITE 1: note = l-Biphenylalanine-4-carboxylic acid
  SITE 3: note = l-phenylalanine-4-carboxylic acid
  SITE 5: note = (2S,4R)-4-aminopyrrolidine-2-carboxylic acid
  SITE 6: note = (2S,3S)-2-amino-3-(4-chloro-1H-indol-3-yl)butanoic acid
  SITE 8: note = d-N-methyl-Alanine
  SITE 10: note = l-Biphenylalanine-4-carboxylic acid
  SITE 12: note = l-2,3-diaminopropionic acid
  SITE 13: note = d-Alanine
  SITE 14: note = l-homoTyrosine
XWXGXXDAGXWXAX

SEQ ID NO: 54 - protein, 14 aa, synthetic construct
  SITE 1: note = l-Biphenylalanine-4-carboxylic acid
  SITE 3: note = l-phenylalanine-4-carboxylic acid
  SITE 5: note = (2S,4R)-4-aminopyrrolidine-2-carboxylic acid
  SITE 6: note = (2S,3S)-2-amino-3-(4-chloro-1H-indol-3-yl)butanoic acid
  SITE 8: note = d-N-methyl-Alanine
  SITE 10: note = l-Biphenylalanine-4-carboxylic acid
  SITE 13: note = d-2,4-diaminobutyric acid
  SITE 14: note = l-homoTyrosine
XWXGXXDAGXWGXX

SEQ ID NO: 55 - protein, 14 aa, synthetic construct
  SITE 1: note = l-Biphenylalanine-4-carboxylic acid
  SITE 3: note = l-phenylalanine-4-carboxylic acid
  SITE 5: note = (2S,4R)-4-aminopyrrolidine-2-carboxylic acid
  SITE 6: note = (2S,3S)-2-amino-3-(4-chloro-1H-indol-3-yl)butanoic acid
  SITE 8: note = d-N-methyl-Alanine
  SITE 10: note = l-Biphenylalanine-4-carboxylic acid
  SITE 13: note = d-2,4-diaminobutyric acid
  SITE 14: note = l-homoTyrosine
XWXGXXEAGXWGXX

SEQ ID NO: 56 - protein, 14 aa, synthetic construct
  SITE 1: note = l-Biphenylalanine-4-carboxylic acid
  SITE 3: note = l-phenylalanine-4-carboxylic acid
  SITE 5: note = (2S,4R)-4-aminopyrrolidine-2-carboxylic acid
  SITE 6: note = (2S,3S)-2-amino-3-(4-chloro-1H-indol-3-yl)butanoic acid
  SITE 8: note = d-N-methyl-Alanine
  SITE 10: note = l-Biphenylalanine-4-carboxylic acid
  SITE 13: note = d-2,4-diaminobutyric acid
  SITE 14: note = l-homoTyrosine
XWXGXXNAGXWGXX

SEQ ID NO: 57 - protein, 14 aa, synthetic construct
  SITE 1: note = l-Biphenylalanine-4-carboxylic acid
  SITE 3: note = l-phenylalanine-4-carboxylic acid
  SITE 5: note = (2S,4R)-4-aminopyrrolidine-2-carboxylic acid
  SITE 6: note = (2S,3S)-2-amino-3-(4-chloro-1H-indol-3-yl)butanoic acid
  SITE 8: note = d-N-methyl-Alanine
  SITE 10: note = l-Biphenylalanine-4-carboxylic acid
  SITE 13: note = d-2,4-diaminobutyric acid
  SITE 14: note = l-homoTyrosine
XWXGXXQAGXWGXX

SEQ ID NO: 58 - protein, 14 aa, synthetic construct
  SITE 1: note = l-Biphenylalanine-4-carboxylic acid
  SITE 3: note = l-phenylalanine-4-carboxylic acid
  SITE 5: note = (2S,4R)-4-aminopyrrolidine-2-carboxylic acid
  SITE 6: note = (2S,3S)-2-amino-3-(4-fluoro-1H-indol-3-yl)butanoic acid
  SITE 8: note = d-N-methyl-Alanine
  SITE 10: note = l-Biphenylalanine-4-carboxylic acid
  SITE 13: note = d-Alanine
  SITE 14: note = l-homoTyrosine
XWXGXXAAGXKLAX

SEQ ID NO: 59 - protein, 14 aa, synthetic construct
  SITE 1: note = l-Biphenylalanine-4-carboxylic acid
  SITE 3: note = l-phenylalanine-4-carboxylic acid
  SITE 5: note = (2S,4R)-4-aminopyrrolidine-2-carboxylic acid
  SITE 6: note = (2S,3S)-2-amino-3-(4-fluoro-1H-indol-3-yl)butanoic acid
  SITE 8: note = d-N-methyl-Alanine
  SITE 10: note = l-Biphenylalanine-4-carboxylic acid
  SITE 11: note = 4-Pyridylalanine
  SITE 13: note = d-Alanine
  SITE 14: note = l-homoTyrosine
XWXGXXDAGXXLAX

SEQ ID NO: 60 - protein, 14 aa, synthetic construct
  SITE 1: note = l-Biphenylalanine-4-carboxylic acid
  SITE 3: note = l-phenylalanine-4-carboxylic acid
  SITE 5: note = (2S,4R)-4-aminopyrrolidine-2-carboxylic acid
  SITE 6: note = (2S,3S)-2-amino-3-(4-fluoro-1H-indol-3-yl)butanoic acid
  SITE 8: note = d-N-methyl-Alanine
  SITE 10: note = l-Biphenylalanine-4-carboxylic acid
  SITE 13: note = d-Alanine
  SITE 14: note = l-homoTyrosine
XWXGXXDAGXFLAX

SEQ ID NO: 61 - protein, 14 aa, synthetic construct
  SITE 1: note = l-Biphenylalanine-4-carboxylic acid
  SITE 3: note = l-phenylalanine-4-carboxylic acid
  SITE 5: note = (2S,4R)-4-aminopyrrolidine-2-carboxylic acid
  SITE 6: note = (2S,3S)-2-amino-3-(4-fluoro-1H-indol-3-yl)butanoic acid
  SITE 8: note = d-N-methyl-Alanine
  SITE 10: note = l-Biphenylalanine-4-carboxylic acid
  SITE 11: note = (S)-2-amino-4-(pyridin-4-yl)butanoic acid
  SITE 13: note = d-Alanine
  SITE 14: note = l-homoTyrosine
XWXGXXDAGXXLAX

SEQ ID NO: 62 - protein, 14 aa, synthetic construct
  SITE 1: note = l-Biphenylalanine-4-carboxylic acid
  SITE 3: note = l-phenylalanine-4-carboxylic acid
  SITE 5: note = (2S,4R)-4-aminopyrrolidine-2-carboxylic acid
  SITE 6: note = (2S,3S)-2-amino-3-(4-fluoro-1H-indol-3-yl)butanoic acid
  SITE 8: note = d-N-methyl-Alanine
  SITE 10: note = l-Biphenylalanine-4-carboxylic acid
  SITE 11: note = l-homoLysine
  SITE 13: note = d-Alanine
  SITE 14: note = l-homoTyrosine
XWXGXXDAGXXLAX

SEQ ID NO: 63 - protein, 14 aa, synthetic construct
  SITE 1: note = l-Biphenylalanine-4-carboxylic acid
  SITE 3: note = l-phenylalanine-4-carboxylic acid
  SITE 5: note = (2S,4R)-4-aminopyrrolidine-2-carboxylic acid
  SITE 6: note = (2S,3S)-2-amino-3-(4-fluoro-1H-indol-3-yl)butanoic acid
  SITE 8: note = d-N-methyl-Alanine
  SITE 10: note = l-Biphenylalanine-4-carboxylic acid
  SITE 11: note = l-homoGlutamine
  SITE 13: note = d-Alanine
  SITE 14: note = l-homoTyrosine
XWXGXXDAGXXLAX

SEQ ID NO: 64 - protein, 14 aa, synthetic construct
  SITE 1: note = l-Biphenylalanine-4-carboxylic acid
  SITE 3: note = l-phenylalanine-4-carboxylic acid
  SITE 5: note = (2S,4R)-4-aminopyrrolidine-2-carboxylic acid
  SITE 6: note = (2S,3S)-2-amino-3-(4-fluoro-1H-indol-3-yl)butanoic acid
  SITE 8: note = d-N-methyl-Alanine
  SITE 10: note = l-Biphenylalanine-4-carboxylic acid
  SITE 12: note = (S)-2-amino-3-(tetrahydro-2H-pyran-4-yl)propanoic acid
  SITE 13: note = d-Alanine
  SITE 14: note = (S)-2-amino-4-(5-cyanopyridin-3-yl)butanoic acid
XWXGXXDAGXKXAX

SEQ ID NO: 65 - protein, 14 aa, synthetic construct
  SITE 1: note = l-Biphenylalanine-4-carboxylic acid
  SITE 3: note = l-phenylalanine-4-carboxylic acid
  SITE 5: note = (2S,4R)-4-aminopyrrolidine-2-carboxylic acid
  SITE 6: note = (2S,3S)-2-amino-3-(4-fluoro-1H-indol-3-yl)butanoic acid
  SITE 8: note = d-N-methyl-Alanine
  SITE 10: note = l-Biphenylalanine-4-carboxylic acid
  SITE 12: note = (S)-2-amino-3-(tetrahydro-2H-pyran-4-yl)propanoic acid
  SITE 13: note = d-Alanine
  SITE 14: note = l-homoTyrosine
XWXGXXDAGXKXAX

SEQ ID NO: 66 - protein, 14 aa, synthetic construct
  SITE 1: note = l-Biphenylalanine-4-carboxylic acid
  SITE 3: note = l-phenylalanine-4-carboxylic acid
  SITE 5: note = (2S,4R)-4-aminopyrrolidine-2-carboxylic acid
  SITE 6: note = (2S,3S)-2-amino-3-(4-fluoro-1H-indol-3-yl)butanoic acid
  SITE 8: note = d-N-methyl-Alanine
  SITE 10: note = l-Biphenylalanine-4-carboxylic acid
  SITE 13: note = d-Alanine
  SITE 14: note = (S)-2-amino-4-(5-cyanopyridin-3-yl)butanoic acid
XWXGXXDAGXKLAX

SEQ ID NO: 67 - protein, 14 aa, synthetic construct
  SITE 1: note = l-Biphenylalanine-4-carboxylic acid
  SITE 3: note = l-phenylalanine-4-carboxylic acid
  SITE 5: note = (2S,4R)-4-aminopyrrolidine-2-carboxylic acid
  SITE 6: note = (2S,3S)-2-amino-3-(4-fluoro-1H-indol-3-yl)butanoic acid
  SITE 8: note = d-N-methyl-Alanine
  SITE 10: note = l-Biphenylalanine-4-carboxylic acid
  SITE 13: note = d-Alanine
  SITE 14: note = l-homoTyrosine
XWXGXXDAGXKLAX

SEQ ID NO: 68 - protein, 14 aa, synthetic construct
  SITE 1: note = l-Biphenylalanine-4-carboxylic acid
  SITE 3: note = l-phenylalanine-4-carboxylic acid
  SITE 5: note = (2S,4R)-4-aminopyrrolidine-2-carboxylic acid
  SITE 6: note = (2S,3S)-2-amino-3-(4-fluoro-1H-indol-3-yl)butanoic acid
  SITE 8: note = d-N-methyl-Alanine
  SITE 10: note = l-Biphenylalanine-4-carboxylic acid
  SITE 13: note = d-2,4-diaminobutyric acid
  SITE 14: note = l-homoTyrosine
XWXGXXDAGXKLXX

SEQ ID NO: 69 - protein, 14 aa, synthetic construct
  SITE 1: note = l-Biphenylalanine-4-carboxylic acid
  SITE 3: note = l-phenylalanine-4-carboxylic acid
  SITE 5: note = (2S,4R)-4-aminopyrrolidine-2-carboxylic acid
  SITE 6: note = (2S,3S)-2-amino-3-(4-fluoro-1H-indol-3-yl)butanoic acid
  SITE 8: note = d-N-methyl-Alanine
  SITE 10: note = l-Biphenylalanine-4-carboxylic acid
  SITE 13: note = d-Serine
  SITE 14: note = l-homoTyrosine
XWXGXXDAGXKLSX

SEQ ID NO: 70 - protein, 14 aa, synthetic construct
  SITE 1: note = l-Biphenylalanine-4-carboxylic acid
  SITE 3: note = l-phenylalanine-4-carboxylic acid
  SITE 5: note = (2S,4R)-4-aminopyrrolidine-2-carboxylic acid
  SITE 6: note = (2S,3S)-2-amino-3-(4-fluoro-1H-indol-3-yl)butanoic acid
  SITE 8: note = d-N-methyl-Alanine
  SITE 10: note = l-Biphenylalanine-4-carboxylic acid
  SITE 14: note = l-homoTyrosine
XWXGXXDAGXKLGX

SEQ ID NO: 71 - protein, 14 aa, synthetic construct
  SITE 1: note = l-Biphenylalanine-4-carboxylic acid
  SITE 3: note = l-phenylalanine-4-carboxylic acid
  SITE 5: note = (2S,4R)-4-aminopyrrolidine-2-carboxylic acid
  SITE 6: note = (2S,3S)-2-amino-3-(4-fluoro-1H-indol-3-yl)butanoic acid
  SITE 8: note = d-N-methyl-Alanine
  SITE 10: note = l-Biphenylalanine-4-carboxylic acid
  SITE 12: note = l-Norvaline
  SITE 13: note = d-Alanine
  SITE 14: note = l-homoTyrosine
XWXGXXDAGXKXAX

SEQ ID NO: 72 - protein, 14 aa, synthetic construct
  SITE 1: note = l-Biphenylalanine-4-carboxylic acid
  SITE 3: note = l-phenylalanine-4-carboxylic acid
  SITE 5: note = (2S,4R)-4-aminopyrrolidine-2-carboxylic acid
  SITE 6: note = (2S,3S)-2-amino-3-(4-fluoro-1H-indol-3-yl)butanoic acid
  SITE 8: note = d-N-methyl-Alanine
  SITE 10: note = l-Biphenylalanine-4-carboxylic acid
  SITE 13: note = d-Alanine
  SITE 14: note = l-homoTyrosine
XWXGXXDAGXKSAX

SEQ ID NO: 73 - protein, 14 aa, synthetic construct
  SITE 1: note = l-Biphenylalanine-4-carboxylic acid
  SITE 3: note = l-phenylalanine-4-carboxylic acid
  SITE 5: note = (2S,4R)-4-aminopyrrolidine-2-carboxylic acid
  SITE 6: note = (2S,3S)-2-amino-3-(4-fluoro-1H-indol-3-yl)butanoic acid
  SITE 8: note = d-N-methyl-Alanine
  SITE 10: note = l-Biphenylalanine-4-carboxylic acid
  SITE 11: note = (S)-2-amino-3-(3-(aminomethyl)phenyl)propanoic acid
  SITE 13: note = d-Alanine
  SITE 14: note = l-homoTyrosine
XWXGXXDAGXXLAX

SEQ ID NO: 74 - protein, 14 aa, synthetic construct
  SITE 1: note = l-Biphenylalanine-4-carboxylic acid
  SITE 3: note = l-phenylalanine-4-carboxylic acid
  SITE 5: note = (2S,4R)-4-aminopyrrolidine-2-carboxylic acid
  SITE 6: note = (2S,3S)-2-amino-3-(4-fluoro-1H-indol-3-yl)butanoic acid
  SITE 8: note = d-N-methyl-Alanine
  SITE 10: note = l-Biphenylalanine-4-carboxylic acid
  SITE 11: note = (S)-2-amino-3-(3-(aminomethyl)phenyl)propanoic acid
  SITE 13: note = d-Alanine
  SITE 14: note = l-homoTyrosine
XWXGXXDAGXXSAX

SEQ ID NO: 75 - protein, 14 aa, synthetic construct
  SITE 1: note = l-Biphenylalanine-4-carboxylic acid
  SITE 3: note = l-phenylalanine-4-carboxylic acid
  SITE 5: note = (2S,4R)-4-aminopyrrolidine-2-carboxylic acid
  SITE 6: note = (2S,3S)-2-amino-3-(4-fluoro-1H-indol-3-yl)butanoic acid
  SITE 8: note = d-N-methyl-Alanine
  SITE 10: note = l-Biphenylalanine-4-carboxylic acid
  SITE 11: note = (S)-2-amino-3-(3-phenylphenyl)propanoic acid
  SITE 13: note = d-Alanine
  SITE 14: note = l-homoTyrosine
XWXGXXDAGXXLAX

SEQ ID NO: 76 - protein, 14 aa, synthetic construct
  SITE 1: note = l-Biphenylalanine-4-carboxylic acid
  SITE 3: note = l-phenylalanine-4-carboxylic acid
  SITE 5: note = (2S,4R)-4-aminopyrrolidine-2-carboxylic acid
  SITE 6: note = (2S,3S)-2-amino-3-(4-fluoro-1H-indol-3-yl)butanoic acid
  SITE 8: note = d-N-methyl-Alanine
  SITE 10: note = l-Biphenylalanine-4-carboxylic acid
  SITE 11: note = (S)-2-amino-3-(3-prop-2-enoxyphenyl)propanoic acid
  SITE 13: note = d-Alanine
  SITE 14: note = l-homoTyrosine
XWXGXXDAGXXLAX

SEQ ID NO: 77 - protein, 14 aa, synthetic construct
  SITE 1: note = l-Biphenylalanine-4-carboxylic acid
  SITE 3: note = l-phenylalanine-4-carboxylic acid
  SITE 5: note = (2S,4R)-4-aminopyrrolidine-2-carboxylic acid
  SITE 6: note = (2S,3S)-2-amino-3-(4-fluoro-1H-indol-3-yl)butanoic acid
  SITE 8: note = d-N-methyl-Alanine
  SITE 10: note = l-Biphenylalanine-4-carboxylic acid
  SITE 13: note = d-2,4-diaminobutyric acid
  SITE 14: note = l-homoTyrosine
XWXGXXDAGXWGXX

SEQ ID NO: 78 - protein, 14 aa, synthetic construct
  SITE 1: note = l-Biphenylalanine-4-carboxylic acid
  SITE 3: note = l-phenylalanine-4-carboxylic acid
  SITE 5: note = (2S,4R)-4-aminopyrrolidine-2-carboxylic acid
  SITE 6: note = (2S,3S)-2-amino-3-(4-fluoro-1H-indol-3-yl)butanoic acid
  SITE 8: note = d-N-methyl-Alanine
  SITE 10: note = l-Biphenylalanine-4-carboxylic acid
  SITE 13: note = d-Alanine
  SITE 14: note = l-homoTyrosine
XWXGXXDAGXWLAX

SEQ ID NO: 79 - protein, 14 aa, synthetic construct
  SITE 1: note = l-Biphenylalanine-4-carboxylic acid
  SITE 3: note = l-phenylalanine-4-carboxylic acid
  SITE 5: note = (2S,4R)-4-aminopyrrolidine-2-carboxylic acid
  SITE 6: note = (2S,3S)-2-amino-3-(4-fluoro-1H-indol-3-yl)butanoic acid
  SITE 8: note = d-N-methyl-Alanine
  SITE 10: note = l-Biphenylalanine-4-carboxylic acid
  SITE 12: note = l-Norvaline
  SITE 13: note = d-Alanine
XWXGXXDAGXWXAA

SEQ ID NO: 80 - protein, 14 aa, synthetic construct
  SITE 1: note = l-Biphenylalanine-4-carboxylic acid
  SITE 3: note = l-phenylalanine-4-carboxylic acid
  SITE 5: note = (2S,4R)-4-aminopyrrolidine-2-carboxylic acid
  SITE 6: note = (2S,3S)-2-amino-3-(4-fluoro-1H-indol-3-yl)butanoic acid
  SITE 8: note = d-N-methyl-Alanine
  SITE 10: note = l-Biphenylalanine-4-carboxylic acid
  SITE 13: note = d-Alanine
  SITE 14: note = l-homoTyrosine
XWXGXXNAGXKLAX

SEQ ID NO: 81 - protein, 14 aa, synthetic construct
  SITE 1: note = l-Biphenylalanine-4-carboxylic acid
  SITE 3: note = l-phenylalanine-4-carboxylic acid
  SITE 5: note = (2S,4R)-4-aminopyrrolidine-2-carboxylic acid
  SITE 6: note = (2S,3S)-2-amino-3-(4-fluoro-1H-indol-3-yl)butanoic acid
  SITE 8: note = d-N-methyl-Alanine
  SITE 10: note = l-Biphenylalanine-4-carboxylic acid
  SITE 13: note = d-2,4-diaminobutyric acid
  SITE 14: note = l-homoTyrosine
XWXGXXNAGXKLXX

SEQ ID NO: 82 - protein, 14 aa, synthetic construct
  SITE 1: note = l-Biphenylalanine-4-carboxylic acid
  SITE 3: note = l-phenylalanine-4-carboxylic acid
  SITE 5: note = (2S,4R)-4-(benzylamino)pyrrolidine-2-carboxylic acid
  SITE 6: note = (2S,3S)-2-amino-3-(naphthalen-1-yl)butanoic acid
  SITE 8: note = d-N-methyl-Alanine
  SITE 10: note = l-Biphenylalanine-4-carboxylic acid
  SITE 12: note = l-2,3-diaminopropionic acid
  SITE 13: note = d-Alanine
  SITE 14: note = l-homoTyrosine
XWXGXXDAGXWXAX

SEQ ID NO: 83 - protein, 14 aa, synthetic construct
  SITE 1: note = l-Biphenylalanine-4-carboxylic acid
  SITE 3: note = l-phenylalanine-4-carboxylic acid
  SITE 5: note = (2S,4R)-4-(phenethylamino)pyrrolidine-2-carboxylic acid
  SITE 6: note = (2S,3S)-2-amino-3-(naphthalen-1-yl)butanoic acid
  SITE 8: note = d-N-methyl-Alanine
  SITE 10: note = l-Biphenylalanine-4-carboxylic acid
  SITE 12: note = l-2,3-diaminopropionic acid
  SITE 13: note = d-Alanine
  SITE 14: note = l-homoTyrosine
XWXGXXDAGXWXAX

SEQ ID NO: 84 - protein, 14 aa, synthetic construct
  SITE 1: note = l-Biphenylalanine-4-carboxylic acid
  SITE 3: note = l-phenylalanine-4-carboxylic acid
  SITE 5: note = (2S,4R)-4-(ethylamino)pyrrolidine-2-carboxylic acid
  SITE 6: note = (2S,3S)-2-amino-3-(naphthalen-1-yl)butanoic acid
  SITE 8: note = d-N-methyl-Alanine
  SITE 10: note = l-Biphenylalanine-4-carboxylic acid
  SITE 12: note = l-2,3-diaminopropionic acid
  SITE 13: note = d-Alanine
  SITE 14: note = l-homoTyrosine
XWXGXXDAGXWXAX

SEQ ID NO: 85 - protein, 14 aa, synthetic construct
  SITE 1: note = (S)-2-amino-3-(4-(4-acetylpiperazin-1-yl)phenyl)propanoic acid
  SITE 3: note = l-phenylalanine-4-carboxylic acid
  SITE 5: note = (2S,4R)-4-aminopyrrolidine-2-carboxylic acid
  SITE 6: note = (2S,3S)-2-amino-3-(4-chloro-1H-indol-3-yl)butanoic acid
  SITE 8: note = d-N-methyl-Alanine
  SITE 10: note = l-Biphenylalanine-4-carboxylic acid
  SITE 13: note = d-2,4-diaminobutyric acid
  SITE 14: note = l-homoTyrosine
XWXGXXDAGXWGXX

SEQ ID NO: 86 - protein, 14 aa, synthetic construct
  SITE 1: note = (S)-2-(4-(2-amino-2-carboxyethyl)phenyl)pyrimidine-5-carboxylic acid
  SITE 3: note = l-phenylalanine-4-carboxylic acid
  SITE 5: note = (2S,4R)-4-aminopyrrolidine-2-carboxylic acid
  SITE 6: note = (2S,3S)-2-amino-3-(naphthalen-1-yl)butanoic acid
  SITE 8: note = d-N-methyl-Alanine
  SITE 10: note = l-Biphenylalanine-4-carboxylic acid
  SITE 12: note = l-2,3-diaminopropionic acid
  SITE 13: note = d-Alanine
  SITE 14: note = l-homoTyrosine
XWXGXXDAGXWXAX

SEQ ID NO: 87 - protein, 14 aa, synthetic construct
  SITE 1: note = (S)-2-(4-(2-amino-2-carboxyethyl)phenyl)pyrimidine-5-carboxylic acid
  SITE 3: note = l-phenylalanine-4-carboxylic acid
  SITE 5: note = (2S,4R)-4-aminopyrrolidine-2-carboxylic acid
  SITE 6: note = (2S,3S)-2-amino-3-(naphthalen-1-yl)butanoic acid
  SITE 8: note = d-N-methyl-Alanine
  SITE 10: note = l-Biphenylalanine-4-carboxylic acid
  SITE 12: note = l-2,3-diaminopropionic acid
  SITE 13: note = d-Alanine
  SITE 14: note = l-homoTyrosine
XWXGXXDAGXWXAX

SEQ ID NO: 88 - protein, 14 aa, synthetic construct
  SITE 1: note = (S)-3-(2-(4-acetylpiperazin-1-yl)pyrimidin-5-yl)-2-aminopropanoic acid
  SITE 3: note = l-phenylalanine-4-carboxylic acid
  SITE 5: note = (2S,4R)-4-aminopyrrolidine-2-carboxylic acid
  SITE 6: note = (2S,3S)-2-amino-3-(naphthalen-1-yl)butanoic acid
  SITE 8: note = d-N-methyl-Alanine
  SITE 10: note = l-Biphenylalanine-4-carboxylic acid
  SITE 12: note = l-2,3-diaminopropionic acid
  SITE 13: note = d-Alanine
  SITE 14: note = l-homoTyrosine
XWXGXXDAGXWXAX

SEQ ID NO: 89 - protein, 14 aa, synthetic construct
  SITE 1: note = l-Tyrosine O-ethyl acetamide
  SITE 3: note = l-phenylalanine-4-carboxylic acid
  SITE 5: note = (2S,4R)-4-aminopyrrolidine-2-carboxylic acid
  SITE 6: note = (2S,3S)-2-amino-3-(naphthalen-1-yl)butanoic acid
  SITE 8: note = d-N-methyl-Alanine
  SITE 10: note = l-Biphenylalanine-4-carboxylic acid
  SITE 12: note = l-2,3-diaminopropionic acid
  SITE 13: note = d-Alanine
  SITE 14: note = l-homoTyrosine
XWXGXXAAGXWXAX

SEQ ID NO: 90 - protein, 14 aa, synthetic construct
  SITE 1: note = l-Tyrosine O-ethyl acetamide
  SITE 3: note = l-phenylalanine-4-carboxylic acid
  SITE 5: note = (2S,4R)-4-aminopyrrolidine-2-carboxylic acid
  SITE 6: note = (2S,3S)-2-amino-3-(naphthalen-1-yl)butanoic acid
  SITE 8: note = d-N-methyl-Alanine
  SITE 10: note = l-Biphenylalanine-4-carboxylic acid
  SITE 11: note = (S)-2-amino-3-(1H-indazol-1-yl)propanoic acid
  SITE 13: note = d-2,4-diaminobutyric acid
  SITE 14: note = (S)-2-amino-4-(5-cyanopyridin-3-yl)butanoic acid
XWXGXXDAGXXGXX

SEQ ID NO: 91 - protein, 14 aa, synthetic construct
  SITE 1: note = l-Tyrosine O-ethyl acetamide
  SITE 3: note = l-phenylalanine-4-carboxylic acid
  SITE 5: note = (2S,4R)-4-aminopyrrolidine-2-carboxylic acid
  SITE 6: note = (2S,3S)-2-amino-3-(naphthalen-1-yl)butanoic acid
  SITE 8: note = d-N-methyl-Alanine
  SITE 10: note = l-Biphenylalanine-4-carboxylic acid
  SITE 11: note = (S)-2-amino-3-(indolin-1-yl)propanoic acid
  SITE 13: note = d-2,4-diaminobutyric acid
  SITE 14: note = (S)-2-amino-4-(5-cyanopyridin-3-yl)butanoic acid
XWXGXXDAGXXGXX

SEQ ID NO: 92 - protein, 14 aa, synthetic construct
  SITE 1: note = l-Tyrosine O-ethyl acetamide
  SITE 3: note = l-phenylalanine-4-carboxylic acid
  SITE 5: note = (2S,4R)-4-aminopyrrolidine-2-carboxylic acid
  SITE 6: note = (2S,3S)-2-amino-3-(naphthalen-1-yl)butanoic acid
  SITE 8: note = d-N-methyl-Alanine
  SITE 10: note = l-Biphenylalanine-4-carboxylic acid
  SITE 11: note = 3-(1-Naphthyl)-l-alanine
  SITE 12: note = l-2,4-diaminobutyric acid
  SITE 13: note = Aminoisobutyric acid
XWXGXXDAGXXXXG

SEQ ID NO: 93 - protein, 14 aa, synthetic construct
  SITE 1: note = l-Tyrosine O-ethyl acetamide
  SITE 3: note = l-phenylalanine-4-carboxylic acid
  SITE 5: note = (2S,4R)-4-aminopyrrolidine-2-carboxylic acid
  SITE 6: note = (2S,3S)-2-amino-3-(naphthalen-1-yl)butanoic acid
  SITE 8: note = d-N-methyl-Alanine
  SITE 10: note = l-Biphenylalanine-4-carboxylic acid
  SITE 11: note = 3-(1-Naphthyl)-l-alanine
  SITE 12: note = l-2,4-diaminobutyric acid
  SITE 13: note = Aminoisobutyric acid
  SITE 14: note = l-homoTyrosine
XWXGXXDAGXXXXX

SEQ ID NO: 94 - protein, 14 aa, synthetic construct
  SITE 1: note = l-Tyrosine O-ethyl acetamide
  SITE 3: note = l-phenylalanine-4-carboxylic acid
  SITE 5: note = (2S,4R)-4-aminopyrrolidine-2-carboxylic acid
  SITE 6: note = (2S,3S)-2-amino-3-(naphthalen-1-yl)butanoic acid
  SITE 8: note = d-N-methyl-Alanine
  SITE 10: note = l-Biphenylalanine-4-carboxylic acid
  SITE 11: note = 3-(1-Naphthyl)-l-alanine
  SITE 12: note = l-2,3-diaminopropionic acid
  SITE 13: note = Aminoisobutyric acid
  SITE 14: note = (S)-2-amino-4-(5-cyanopyridin-3-yl)butanoic acid
XWXGXXDAGXXXXX

SEQ ID NO: 95 - protein, 14 aa, synthetic construct
  SITE 1: note = l-Tyrosine O-ethyl acetamide
  SITE 3: note = l-phenylalanine-4-carboxylic acid
  SITE 5: note = (2S,4R)-4-aminopyrrolidine-2-carboxylic acid
  SITE 6: note = (2S,3S)-2-amino-3-(naphthalen-1-yl)butanoic acid
  SITE 8: note = d-N-methyl-Alanine
  SITE 10: note = l-Biphenylalanine-4-carboxylic acid
  SITE 11: note = 3-(1-Naphthyl)-l-alanine
  SITE 13: note = Aminoisobutyric acid
XWXGXXDAGXXLXG

SEQ ID NO: 96 - protein, 14 aa, synthetic construct
  SITE 1: note = l-Tyrosine O-ethyl acetamide
  SITE 3: note = l-phenylalanine-4-carboxylic acid
  SITE 5: note = (2S,4R)-4-aminopyrrolidine-2-carboxylic acid
  SITE 6: note = (2S,3S)-2-amino-3-(naphthalen-1-yl)butanoic acid
  SITE 8: note = d-N-methyl-Alanine
  SITE 10: note = l-Biphenylalanine-4-carboxylic acid
  SITE 11: note = 3-(1-Naphthyl)-l-alanine
  SITE 13: note = Aminoisobutyric acid
  SITE 14: note = l-homoTyrosine
XWXGXXDAGXXLXX

SEQ ID NO: 97 - protein, 14 aa, synthetic construct
  SITE 1: note = l-Tyrosine O-ethyl acetamide
  SITE 3: note = l-phenylalanine-4-carboxylic acid
  SITE 5: note = (2S,4R)-4-aminopyrrolidine-2-carboxylic acid
  SITE 6: note = (2S,3S)-2-amino-3-(naphthalen-1-yl)butanoic acid
  SITE 8: note = d-N-methyl-Alanine
  SITE 10: note = l-Biphenylalanine-4-carboxylic acid
  SITE 11: note = 3-(1-Naphthyl)-l-alanine
  SITE 13: note = d-Alanine
XWXGXXDAGXXLAA

SEQ ID NO: 98 - protein, 14 aa, synthetic construct
  SITE 1: note = l-Tyrosine O-ethyl acetamide
  SITE 3: note = l-phenylalanine-4-carboxylic acid
  SITE 5: note = (2S,4R)-4-aminopyrrolidine-2-carboxylic acid
  SITE 6: note = (2S,3S)-2-amino-3-(naphthalen-1-yl)butanoic acid
  SITE 8: note = d-N-methyl-Alanine
  SITE 10: note = l-Biphenylalanine-4-carboxylic acid
  SITE 11: note = 3-(1-Naphthyl)-l-alanine
  SITE 12: note = l-Norvaline
  SITE 13: note = d-Alanine
XWXGXXDAGXXXAA

SEQ ID NO: 99 - protein, 14 aa, synthetic construct
  SITE 1: note = l-Tyrosine O-ethyl acetamide
  SITE 3: note = l-phenylalanine-4-carboxylic acid
  SITE 5: note = (2S,4R)-4-aminopyrrolidine-2-carboxylic acid
  SITE 6: note = (2S,3S)-2-amino-3-(naphthalen-1-yl)butanoic acid
  SITE 8: note = d-N-methyl-Alanine
  SITE 10: note = l-Biphenylalanine-4-carboxylic acid
  SITE 11: note = 3-(1-Naphthyl)-l-alanine
  SITE 12: note = l-Ornithine
  SITE 13: note = Aminoisobutyric acid
  SITE 14: note = l-homoTyrosine
XWXGXXDAGXXXXX

SEQ ID NO: 100 - protein, 14 aa, synthetic construct
  SITE 1: note = l-Tyrosine O-ethyl acetamide
  SITE 3: note = l-phenylalanine-4-carboxylic acid
  SITE 5: note = (2S,4R)-4-aminopyrrolidine-2-carboxylic acid
  SITE 6: note = (2S,3S)-2-amino-3-(naphthalen-1-yl)butanoic acid
  SITE 8: note = d-N-methyl-Alanine
  SITE 10: note = l-Biphenylalanine-4-carboxylic acid
  SITE 11: note = 4-Pyridylalanine
  SITE 12: note = l-2,4-diaminobutyric acid
  SITE 13: note = d-Alanine
  SITE 14: note = (S)-2-amino-4-(4-(trifluoromethyl)phenyl)butanoic acid
XWXGXXDAGXXXAX

SEQ ID NO: 101 - protein, 14 aa, synthetic construct
  SITE 1: note = l-Tyrosine O-ethyl acetamide
  SITE 3: note = l-phenylalanine-4-carboxylic acid
  SITE 5: note = (2S,4R)-4-aminopyrrolidine-2-carboxylic acid
  SITE 6: note = (2S,3S)-2-amino-3-(naphthalen-1-yl)butanoic acid
  SITE 8: note = d-N-methyl-Alanine
  SITE 10: note = l-Biphenylalanine-4-carboxylic acid
  SITE 11: note = 4-Pyridylalanine
  SITE 12: note = l-2,4-diaminobutyric acid
  SITE 13: note = d-Alanine
  SITE 14: note = l-homoTyrosine
XWXGXXDAGXXXAX

SEQ ID NO: 102 - protein, 14 aa, synthetic construct
  SITE 1: note = l-Tyrosine O-ethyl acetamide
  SITE 3: note = l-phenylalanine-4-carboxylic acid
  SITE 5: note = (2S,4R)-4-aminopyrrolidine-2-carboxylic acid
  SITE 6: note = (2S,3S)-2-amino-3-(naphthalen-1-yl)butanoic acid
  SITE 8: note = d-N-methyl-Alanine
  SITE 10: note = l-Biphenylalanine-4-carboxylic acid
  SITE 11: note = 4-Pyridylalanine
  SITE 13: note = d-2,4-diaminobutyric acid
  SITE 14: note = (S)-2-amino-4-(5-cyanopyridin-3-yl)butanoic acid
XWXGXXDAGXXGXX

SEQ ID NO: 103 - protein, 14 aa, synthetic construct
  SITE 1: note = l-Tyrosine O-ethyl acetamide
  SITE 3: note = l-phenylalanine-4-carboxylic acid
  SITE 5: note = (2S,4R)-4-aminopyrrolidine-2-carboxylic acid
  SITE 6: note = (2S,3S)-2-amino-3-(naphthalen-1-yl)butanoic acid
  SITE 8: note = d-N-methyl-Alanine
  SITE 10: note = l-Biphenylalanine-4-carboxylic acid
  SITE 11: note = 4-Pyridylalanine
  SITE 13: note = d-Alanine
  SITE 14: note = (S)-2-amino-4-(2-(trifluoromethyl)phenyl)butanoic acid
XWXGXXDAGXXSAX

SEQ ID NO: 104 - protein, 14 aa, synthetic construct
  SITE 1: note = l-Tyrosine O-ethyl acetamide
  SITE 3: note = l-phenylalanine-4-carboxylic acid
  SITE 5: note = (2S,4R)-4-aminopyrrolidine-2-carboxylic acid
  SITE 6: note = (2S,3S)-2-amino-3-(naphthalen-1-yl)butanoic acid
  SITE 8: note = d-N-methyl-Alanine
  SITE 10: note = l-Biphenylalanine-4-carboxylic acid
  SITE 11: note = 4-Pyridylalanine
  SITE 13: note = d-Alanine
  SITE 14: note = (S)-2-amino-4-(3-(trifluoromethyl)phenyl)butanoic acid
XWXGXXDAGXXSAX

SEQ ID NO: 105 - protein, 14 aa, synthetic construct
  SITE 1: note = l-Tyrosine O-ethyl acetamide
  SITE 3: note = l-phenylalanine-4-carboxylic acid
  SITE 5: note = (2S,4R)-4-aminopyrrolidine-2-carboxylic acid
  SITE 6: note = (2S,3S)-2-amino-3-(naphthalen-1-yl)butanoic acid
  SITE 8: note = d-N-methyl-Alanine
  SITE 10: note = l-Biphenylalanine-4-carboxylic acid
  SITE 11: note = 4-Pyridylalanine
  SITE 13: note = d-Alanine
  SITE 14: note = (S)-2-amino-4-(4-(trifluoromethyl)phenyl)butanoic acid
XWXGXXDAGXXSAX

SEQ ID NO: 106 - protein, 14 aa, synthetic construct
  SITE 1: note = l-Tyrosine O-ethyl acetamide
  SITE 3: note = l-phenylalanine-4-carboxylic acid
  SITE 5: note = (2S,4R)-4-aminopyrrolidine-2-carboxylic acid
  SITE 6: note = (2S,3S)-2-amino-3-(naphthalen-1-yl)butanoic acid
  SITE 8: note = d-N-methyl-Alanine
  SITE 10: note = l-Biphenylalanine-4-carboxylic acid
  SITE 11: note = (S)-2-amino-3-(tetrahydro-2H-pyran-4-yl)propanoic acid
  SITE 13: note = d-2,4-diaminobutyric acid
  SITE 14: note = (S)-2-amino-4-(5-cyanopyridin-3-yl)butanoic acid
XWXGXXDAGXXGXX

SEQ ID NO: 107 - protein, 14 aa, synthetic construct
  SITE 1: note = l-Tyrosine O-ethyl acetamide
  SITE 3: note = l-phenylalanine-4-carboxylic acid
  SITE 5: note = (2S,4R)-4-aminopyrrolidine-2-carboxylic acid
  SITE 6: note = (2S,3S)-2-amino-3-(naphthalen-1-yl)butanoic acid
  SITE 8: note = d-N-methyl-Alanine
  SITE 10: note = l-Biphenylalanine-4-carboxylic acid
  SITE 13: note = Aminoisobutyric acid
  SITE 14: note = l-homoTyrosine
XWXGXXDAGXKGXX

SEQ ID NO: 108 - protein, 14 aa, synthetic construct
  SITE 1: note = l-Tyrosine O-ethyl acetamide
  SITE 3: note = l-phenylalanine-4-carboxylic acid
  SITE 5: note = (2S,4R)-4-aminopyrrolidine-2-carboxylic acid
  SITE 6: note = (2S,3S)-2-amino-3-(naphthalen-1-yl)butanoic acid
  SITE 8: note = d-N-methyl-Alanine
  SITE 10: note = l-Biphenylalanine-4-carboxylic acid
  SITE 13: note = d-Alanine
  SITE 14: note = l-homoTyrosine
XWXGXXDAGXKGAX

SEQ ID NO: 109 - protein, 14 aa, synthetic construct
  SITE 1: note = l-Tyrosine O-ethyl acetamide
  SITE 3: note = l-phenylalanine-4-carboxylic acid
  SITE 5: note = (2S,4R)-4-aminopyrrolidine-2-carboxylic acid
  SITE 6: note = (2S,3S)-2-amino-3-(naphthalen-1-yl)butanoic acid
  SITE 8: note = d-N-methyl-Alanine
  SITE 10: note = l-Biphenylalanine-4-carboxylic acid
  SITE 13: note = d-N-methyl-Alanine
  SITE 14: note = l-homoTyrosine
XWXGXXDAGXKGAX

SEQ ID NO: 110 - protein, 14 aa, synthetic construct
  SITE 1: note = l-Tyrosine O-ethyl acetamide
  SITE 3: note = l-phenylalanine-4-carboxylic acid
  SITE 5: note = (2S,4R)-4-aminopyrrolidine-2-carboxylic acid
  SITE 6: note = (2S,3S)-2-amino-3-(naphthalen-1-yl)butanoic acid
  SITE 8: note = d-N-methyl-Alanine
  SITE 10: note = l-Biphenylalanine-4-carboxylic acid
  SITE 13: note = d-Alanine
  SITE 14: note = l-homoTyrosine
XWXGXXDAGXKLAX

SEQ ID NO: 111 - protein, 14 aa, synthetic construct
  SITE 1: note = l-Tyrosine O-ethyl acetamide
  SITE 3: note = l-phenylalanine-4-carboxylic acid
  SITE 5: note = (2S,4R)-4-aminopyrrolidine-2-carboxylic acid
  SITE 6: note = (2S,3S)-2-amino-3-(naphthalen-1-yl)butanoic acid
  SITE 8: note = d-N-methyl-Alanine
  SITE 10: note = l-Biphenylalanine-4-carboxylic acid
  SITE 13: note = d-Alanine
  SITE 14: note = (S)-2-amino-4-(4-(trifluoromethyl)phenyl)butanoic acid
XWXGXXDAGXKSAX

SEQ ID NO: 112 - protein, 14 aa, synthetic construct
  SITE 1: note = l-Tyrosine O-ethyl acetamide
  SITE 3: note = l-phenylalanine-4-carboxylic acid
  SITE 5: note = (2S,4R)-4-aminopyrrolidine-2-carboxylic acid
  SITE 6: note = (2S,3S)-2-amino-3-(naphthalen-1-yl)butanoic acid
  SITE 8: note = d-N-methyl-Alanine
  SITE 10: note = l-Biphenylalanine-4-carboxylic acid
  SITE 13: note = d-Alanine
  SITE 14: note = l-homoTyrosine
XWXGXXDAGXKSAX

SEQ ID NO: 113 - protein, 14 aa, synthetic construct
  SITE 1: note = l-Tyrosine O-ethyl acetamide
  SITE 3: note = l-phenylalanine-4-carboxylic acid
  SITE 5: note = (2S,4R)-4-aminopyrrolidine-2-carboxylic acid
  SITE 6: note = (2S,3S)-2-amino-3-(naphthalen-1-yl)butanoic acid
  SITE 8: note = d-N-methyl-Alanine
  SITE 10: note = l-Biphenylalanine-4-carboxylic acid
  SITE 11: note = (S)-2-amino-3-(pyrimidin-5-yl)propanoic acid
  SITE 13: note = d-2,4-diaminobutyric acid
  SITE 14: note = (S)-2-amino-4-(5-cyanopyridin-3-yl)butanoic acid
XWXGXXDAGXXGXX

SEQ ID NO: 114 - protein, 14 aa, synthetic construct
  SITE 1: note = l-Tyrosine O-ethyl acetamide
  SITE 3: note = l-phenylalanine-4-carboxylic acid
  SITE 5: note = (2S,4R)-4-aminopyrrolidine-2-carboxylic acid
  SITE 6: note = (2S,3S)-2-amino-3-(naphthalen-1-yl)butanoic acid
  SITE 8: note = d-N-methyl-Alanine
  SITE 10: note = l-Biphenylalanine-4-carboxylic acid
  SITE 11: note = (S)-2-amino-3-(1H-pyrrolo[2,3-b]pyridin-3-yl)propanoic acid
  SITE 13: note = d-2,4-diaminobutyric acid
  SITE 14: note = (S)-2-amino-4-(5-cyanopyridin-3-yl)butanoic acid
XWXGXXDAGXXGXX

SEQ ID NO: 115 - protein, 14 aa, synthetic construct
  SITE 1: note = l-Tyrosine O-ethyl acetamide
  SITE 3: note = l-phenylalanine-4-carboxylic acid
  SITE 5: note = (2S,4R)-4-aminopyrrolidine-2-carboxylic acid
  SITE 6: note = (2S,3S)-2-amino-3-(naphthalen-1-yl)butanoic acid
  SITE 8: note = d-N-methyl-Alanine
  SITE 10: note = l-Biphenylalanine-4-carboxylic acid
  SITE 12: note = l-2,4-diaminobutyric acid
  SITE 13: note = d-Alanine
  SITE 14: note = l-homoPhenylalanine
XWXGXXDAGXWXAX

SEQ ID NO: 116 - protein, 14 aa, synthetic construct
  SITE 1: note = l-Tyrosine O-ethyl acetamide
  SITE 3: note = l-phenylalanine-4-carboxylic acid
  SITE 5: note = (2S,4R)-4-aminopyrrolidine-2-carboxylic acid
  SITE 6: note = (2S,3S)-2-amino-3-(naphthalen-1-yl)butanoic acid
  SITE 8: note = d-N-methyl-Alanine
  SITE 10: note = l-Biphenylalanine-4-carboxylic acid
  SITE 12: note = l-2,4-diaminobutyric acid
  SITE 13: note = d-Alanine
  SITE 14: note = l-homoTyrosine
XWXGXXDAGXWXAX

SEQ ID NO: 117 - protein, 14 aa, synthetic construct
  SITE 1: note = l-Tyrosine O-ethyl acetamide
  SITE 3: note = l-phenylalanine-4-carboxylic acid
  SITE 5: note = (2S,4R)-4-aminopyrrolidine-2-carboxylic acid
  SITE 6: note = (2S,3S)-2-amino-3-(naphthalen-1-yl)butanoic acid
  SITE 8: note = d-N-methyl-Alanine
  SITE 10: note = l-Biphenylalanine-4-carboxylic acid
  SITE 12: note = l-2,3-diaminopropionic acid
  SITE 13: note = Aminoisobutyric acid
  SITE 14: note = l-homoTyrosine
XWXGXXDAGXWXXX

SEQ ID NO: 118 - protein, 14 aa, synthetic construct
  SITE 1: note = l-Tyrosine O-ethyl acetamide
  SITE 3: note = l-phenylalanine-4-carboxylic acid
  SITE 5: note = (2S,4R)-4-aminopyrrolidine-2-carboxylic acid
  SITE 6: note = (2S,3S)-2-amino-3-(naphthalen-1-yl)butanoic acid
  SITE 8: note = d-N-methyl-Alanine
  SITE 10: note = l-Biphenylalanine-4-carboxylic acid
  SITE 12: note = l-2,3-diaminopropionic acid
  SITE 13: note = d-Alanine
XWXGXXDAGXWXAA

SEQ ID NO: 119 - protein, 14 aa, synthetic construct
  SITE 1: note = l-Tyrosine O-ethyl acetamide
  SITE 3: note = l-phenylalanine-4-carboxylic acid
  SITE 5: note = (2S,4R)-4-aminopyrrolidine-2-carboxylic acid
  SITE 6: note = (2S,3S)-2-amino-3-(naphthalen-1-yl)butanoic acid
  SITE 8: note = d-N-methyl-Alanine
  SITE 10: note = l-Biphenylalanine-4-carboxylic acid
  SITE 12: note = l-2,3-diaminopropionic acid
  SITE 13: note = d-Alanine
  SITE 14: note = l-homoTyrosine
XWXGXXDAGXWXAX

SEQ ID NO: 120 - protein, 14 aa, synthetic construct
  SITE 1: note = l-Tyrosine O-ethyl acetamide
  SITE 3: note = l-phenylalanine-4-carboxylic acid
  SITE 5: note = (2S,4R)-4-aminopyrrolidine-2-carboxylic acid
  SITE 6: note = (2S,3S)-2-amino-3-(naphthalen-1-yl)butanoic acid
  SITE 8: note = d-N-methyl-Alanine
  SITE 10: note = l-Biphenylalanine-4-carboxylic acid
  SITE 12: note = l-2,3-diaminopropionic acid
  SITE 13: note = d-Alanine
  SITE 14: note = (S)-2-amino-3-(4-(2-morpholinoethoxy)phenyl)propanoic acid
XWXGXXDAGXWXAX

SEQ ID NO: 121 - protein, 14 aa, synthetic construct
  SITE 1: note = l-Tyrosine O-ethyl acetamide
  SITE 3: note = l-phenylalanine-4-carboxylic acid
  SITE 5: note = (2S,4R)-4-aminopyrrolidine-2-carboxylic acid
  SITE 6: note = (2S,3S)-2-amino-3-(naphthalen-1-yl)butanoic acid
  SITE 8: note = d-N-methyl-Alanine
  SITE 10: note = l-Biphenylalanine-4-carboxylic acid
  SITE 12: note = l-2,3-diaminopropionic acid
  SITE 13: note = d-N-methyl-Alanine
  SITE 14: note = l-homoTyrosine
XWXGXXDAGXWXAX

SEQ ID NO: 122 - protein, 14 aa, synthetic construct
  SITE 1: note = l-Tyrosine O-ethyl acetamide
  SITE 3: note = l-phenylalanine-4-carboxylic acid
  SITE 5: note = (2S,4R)-4-aminopyrrolidine-2-carboxylic acid
  SITE 6: note = (2S,3S)-2-amino-3-(naphthalen-1-yl)butanoic acid
  SITE 8: note = d-N-methyl-Alanine
  SITE 10: note = l-Biphenylalanine-4-carboxylic acid
  SITE 13: note = d-2,4-diaminobutyric acid
  SITE 14: note = (S)-2-amino-4-(5-cyanopyridin-3-yl)butanoic acid
XWXGXXDAGXWGXX

SEQ ID NO: 123 - protein, 14 aa, synthetic construct
  SITE 1: note = l-Tyrosine O-ethyl acetamide
  SITE 3: note = l-phenylalanine-4-carboxylic acid
  SITE 5: note = (2S,4R)-4-aminopyrrolidine-2-carboxylic acid
  SITE 6: note = (2S,3S)-2-amino-3-(naphthalen-1-yl)butanoic acid
  SITE 8: note = d-N-methyl-Alanine
  SITE 10: note = l-Biphenylalanine-4-carboxylic acid
  SITE 13: note = d-2,4-diaminobutyric acid
  SITE 14: note = l-homoTyrosine
XWXGXXDAGXWGXX

SEQ ID NO: 124 - protein, 14 aa, synthetic construct
  SITE 1: note = l-Tyrosine O-ethyl acetamide
  SITE 3: note = l-phenylalanine-4-carboxylic acid
  SITE 5: note = (2S,4R)-4-aminopyrrolidine-2-carboxylic acid
  SITE 6: note = (2S,3S)-2-amino-3-(naphthalen-1-yl)butanoic acid
  SITE 8: note = d-N-methyl-Alanine
  SITE 10: note = l-Biphenylalanine-4-carboxylic acid
  SITE 13: note = d-Alanine
XWXGXXDAGXWLAA

SEQ ID NO: 125 - protein, 14 aa, synthetic construct
  SITE 1: note = l-Tyrosine O-ethyl acetamide
  SITE 3: note = l-phenylalanine-4-carboxylic acid
  SITE 5: note = (2S,4R)-4-aminopyrrolidine-2-carboxylic acid
  SITE 6: note = (2S,3S)-2-amino-3-(naphthalen-1-yl)butanoic acid
  SITE 8: note = d-N-methyl-Alanine
  SITE 10: note = l-Biphenylalanine-4-carboxylic acid
  SITE 13: note = d-Alanine
  SITE 14: note = l-homoTyrosine
XWXGXXDAGXWLAX

SEQ ID NO: 126 - protein, 14 aa, synthetic construct
  SITE 1: note = l-Tyrosine O-ethyl acetamide
  SITE 3: note = l-phenylalanine-4-carboxylic acid
  SITE 5: note = (2S,4R)-4-aminopyrrolidine-2-carboxylic acid
  SITE 6: note = (2S,3S)-2-amino-3-(naphthalen-1-yl)butanoic acid
  SITE 8: note = d-N-methyl-Alanine
  SITE 10: note = l-Biphenylalanine-4-carboxylic acid
  SITE 13: note = d-2,4-diaminobutyric acid
  SITE 14: note = l-homoTyrosine
XWXGXXDAGXWLXX

SEQ ID NO: 127 - protein, 14 aa, synthetic construct
  SITE 1: note = l-Tyrosine O-ethyl acetamide
  SITE 3: note = l-phenylalanine-4-carboxylic acid
  SITE 5: note = (2S,4R)-4-aminopyrrolidine-2-carboxylic acid
  SITE 6: note = (2S,3S)-2-amino-3-(naphthalen-1-yl)butanoic acid
  SITE 8: note = d-N-methyl-Alanine
  SITE 10: note = l-Biphenylalanine-4-carboxylic acid
  SITE 12: note = l-Ornithine
  SITE 13: note = Aminoisobutyric acid
  SITE 14: note = l-homoTyrosine
XWXGXXDAGXWXXX

SEQ ID NO: 128 - protein, 14 aa, synthetic construct
  SITE 1: note = l-Tyrosine O-ethyl acetamide
  SITE 3: note = l-phenylalanine-4-carboxylic acid
  SITE 5: note = (2S,4R)-4-aminopyrrolidine-2-carboxylic acid
  SITE 6: note = (2S,3S)-2-amino-3-(naphthalen-1-yl)butanoic acid
  SITE 8: note = d-N-methyl-Alanine
  SITE 10: note = l-Biphenylalanine-4-carboxylic acid
  SITE 13: note = d-Alanine
  SITE 14: note = l-homoTyrosine
XWXGXXDAGXWSAX

SEQ ID NO: 129 - protein, 14 aa, synthetic construct
  SITE 1: note = l-Tyrosine O-ethyl acetamide
  SITE 3: note = l-phenylalanine-4-carboxylic acid
  SITE 5: note = (2S,4R)-4-aminopyrrolidine-2-carboxylic acid
  SITE 6: note = (2S,3S)-2-amino-3-(naphthalen-1-yl)butanoic acid
  SITE 8: note = d-N-methyl-Alanine
  SITE 10: note = l-Biphenylalanine-4-carboxylic acid
  SITE 12: note = l-2,3-diaminopropionic acid
  SITE 13: note = d-Alanine
  SITE 14: note = l-homoTyrosine
XWXGXXNAGXWXAX

SEQ ID NO: 130 - protein, 14 aa, synthetic construct
  SITE 1: note = l-Tyrosine O-ethyl acetamide
  SITE 3: note = l-phenylalanine-4-carboxylic acid
  SITE 5: note = (2S,4R)-4-aminopyrrolidine-2-carboxylic acid
  SITE 6: note = (2S,3S)-2-amino-3-(4-chloro-1H-indol-3-yl)butanoic acid
  SITE 8: note = d-N-methyl-Alanine
  SITE 10: note = l-Biphenylalanine-4-carboxylic acid
  SITE 11: note = 3-(1-Naphthyl)-l-alanine
  SITE 12: note = l-2,3-diaminopropionic acid
  SITE 13: note = Aminoisobutyric acid
  SITE 14: note = (S)-2-amino-4-(5-cyanopyridin-3-yl)butanoic acid
XWXGXXDAGXXXXX

SEQ ID NO: 131 - protein, 14 aa, synthetic construct
  SITE 1: note = l-Tyrosine O-ethyl acetamide
  SITE 3: note = l-phenylalanine-4-carboxylic acid
  SITE 5: note = (2S,4R)-4-aminopyrrolidine-2-carboxylic acid
  SITE 6: note = (2S,3S)-2-amino-3-(4-chloro-1H-indol-3-yl)butanoic acid
  SITE 8: note = d-N-methyl-Alanine
  SITE 10: note = l-Biphenylalanine-4-carboxylic acid
  SITE 11: note = 3-(1-Naphthyl)-l-alanine
  SITE 13: note = d-Alanine
  SITE 14: note = l-homoTyrosine
XWXGXXDAGXXLAX

SEQ ID NO: 132 - protein, 14 aa, synthetic construct
  SITE 1: note = l-Tyrosine O-ethyl acetamide
  SITE 3: note = l-phenylalanine-4-carboxylic acid
  SITE 5: note = (2S,4R)-4-aminopyrrolidine-2-carboxylic acid
  SITE 6: note = (2S,3S)-2-amino-3-(4-chloro-1H-indol-3-yl)butanoic acid
  SITE 8: note = d-N-methyl-Alanine
  SITE 10: note = l-Biphenylalanine-4-carboxylic acid
  SITE 11: note = 3-(1-Naphthyl)-l-alanine
  SITE 12: note = l-Ornithine
  SITE 13: note = Aminoisobutyric acid
XWXGXXDAGXXXXG

SEQ ID NO: 133 - protein, 14 aa, synthetic construct
  SITE 1: note = l-Tyrosine O-ethyl acetamide
  SITE 3: note = l-phenylalanine-4-carboxylic acid
  SITE 5: note = (2S,4R)-4-aminopyrrolidine-2-carboxylic acid
  SITE 6: note = (2S,3S)-2-amino-3-(4-chloro-1H-indol-3-yl)butanoic acid
  SITE 8: note = d-N-methyl-Alanine
  SITE 10: note = l-Biphenylalanine-4-carboxylic acid
  SITE 11: note = 3-(1-Naphthyl)-l-alanine
  SITE 13: note = d-Alanine
  SITE 14: note = (S)-2-amino-3-(4-aminophenyl)propanoic acid
XWXGXXDAGXXSAX

SEQ ID NO: 134 - protein, 14 aa, synthetic construct
  SITE 1: note = l-Tyrosine O-ethyl acetamide
  SITE 3: note = l-phenylalanine-4-carboxylic acid
  SITE 5: note = (2S,4R)-4-aminopyrrolidine-2-carboxylic acid
  SITE 6: note = (2S,3S)-2-amino-3-(4-chloro-1H-indol-3-yl)butanoic acid
  SITE 8: note = d-N-methyl-Alanine
  SITE 10: note = l-Biphenylalanine-4-carboxylic acid
  SITE 11: note = 4-Pyridylalanine
  SITE 12: note = l-2,4-diaminobutyric acid
  SITE 13: note = d-Alanine
  SITE 14: note = l-homoTyrosine
XWXGXXDAGXXXAX

SEQ ID NO: 135 - protein, 14 aa, synthetic construct
  SITE 1: note = l-Tyrosine O-ethyl acetamide
  SITE 3: note = l-phenylalanine-4-carboxylic acid
  SITE 5: note = (2S,4R)-4-aminopyrrolidine-2-carboxylic acid
  SITE 6: note = (2S,3S)-2-amino-3-(4-chloro-1H-indol-3-yl)butanoic acid
  SITE 8: note = d-N-methyl-Alanine
  SITE 10: note = l-Biphenylalanine-4-carboxylic acid
  SITE 11: note = 4-Pyridylalanine
  SITE 13: note = d-Alanine
  SITE 14: note = l-homoTyrosine
XWXGXXDAGXXLAX

SEQ ID NO: 136 - protein, 14 aa, synthetic construct
  SITE 1: note = l-Tyrosine O-ethyl acetamide
  SITE 3: note = l-phenylalanine-4-carboxylic acid
  SITE 5: note = (2S,4R)-4-aminopyrrolidine-2-carboxylic acid
  SITE 6: note = (2S,3S)-2-amino-3-(4-chloro-1H-indol-3-yl)butanoic acid
  SITE 8: note = d-N-methyl-Alanine
  SITE 10: note = l-Biphenylalanine-4-carboxylic acid
  SITE 11: note = 4-Pyridylalanine
  SITE 12: note = l-Norvaline
  SITE 13: note = d-Alanine
  SITE 14: note = (S)-2-amino-3-(4,4-difluorocyclohexyl)propanoic acid
XWXGXXDAGXXXAX

SEQ ID NO: 137 - protein, 14 aa, synthetic construct
  SITE 1: note = l-Tyrosine O-ethyl acetamide
  SITE 3: note = l-phenylalanine-4-carboxylic acid
  SITE 5: note = (2S,4R)-4-aminopyrrolidine-2-carboxylic acid
  SITE 6: note = (2S,3S)-2-amino-3-(4-chloro-1H-indol-3-yl)butanoic acid
  SITE 8: note = d-N-methyl-Alanine
  SITE 10: note = l-Biphenylalanine-4-carboxylic acid
  SITE 13: note = d-Alanine
  SITE 14: note = (S)-2-amino-4-(3-(trifluoromethyl)phenyl)butanoic acid
XWXGXXDAGXKLAX

SEQ ID NO: 138 - protein, 14 aa, synthetic construct
  SITE 1: note = l-Tyrosine O-ethyl acetamide
  SITE 3: note = l-phenylalanine-4-carboxylic acid
  SITE 5: note = (2S,4R)-4-aminopyrrolidine-2-carboxylic acid
  SITE 6: note = (2S,3S)-2-amino-3-(4-chloro-1H-indol-3-yl)butanoic acid
  SITE 8: note = d-N-methyl-Alanine
  SITE 10: note = l-Biphenylalanine-4-carboxylic acid
  SITE 13: note = d-Alanine
  SITE 14: note = l-homoTyrosine
XWXGXXDAGXKSAX

SEQ ID NO: 139 - protein, 14 aa, synthetic construct
  SITE 1: note = l-Tyrosine O-ethyl acetamide
  SITE 3: note = l-phenylalanine-4-carboxylic acid
  SITE 5: note = (2S,4R)-4-aminopyrrolidine-2-carboxylic acid
  SITE 6: note = (2S,3S)-2-amino-3-(4-chloro-1H-indol-3-yl)butanoic acid
  SITE 8: note = d-N-methyl-Alanine
  SITE 10: note = l-Biphenylalanine-4-carboxylic acid
  SITE 13: note = d-2,4-diaminobutyric acid
  SITE 14: note = l-homoTyrosine
XWXGXXDAGXKSXX

SEQ ID NO: 140 - protein, 14 aa, synthetic construct
  SITE 1: note = l-Tyrosine O-ethyl acetamide
  SITE 3: note = l-phenylalanine-4-carboxylic acid
  SITE 5: note = (2S,4R)-4-aminopyrrolidine-2-carboxylic acid
  SITE 6: note = (2S,3S)-2-amino-3-(4-chloro-1H-indol-3-yl)butanoic acid
  SITE 8: note = d-N-methyl-Alanine
  SITE 10: note = l-Biphenylalanine-4-carboxylic acid
  SITE 12: note = (S)-2-amino-4-morpholinobutanoic acid
  SITE 13: note = d-Alanine
XWXGXXDAGXWXAG

SEQ ID NO: 141 - protein, 14 aa, synthetic construct
  SITE 1: note = l-Tyrosine O-ethyl acetamide
  SITE 3: note = l-phenylalanine-4-carboxylic acid
  SITE 5: note = (2S,4R)-4-aminopyrrolidine-2-carboxylic acid
  SITE 6: note = (2S,3S)-2-amino-3-(4-chloro-1H-indol-3-yl)butanoic acid
  SITE 8: note = d-N-methyl-Alanine
  SITE 10: note = l-Biphenylalanine-4-carboxylic acid
  SITE 12: note = (S)-2-amino-4-morpholinobutanoic acid
  SITE 13: note = d-Alanine
  SITE 14: note = l-homoTyrosine
XWXGXXDAGXWXAX

SEQ ID NO: 142 - protein, 14 aa, synthetic construct
  SITE 1: note = l-Tyrosine O-ethyl acetamide
  SITE 3: note = l-phenylalanine-4-carboxylic acid
  SITE 5: note = (2S,4R)-4-aminopyrrolidine-2-carboxylic acid
  SITE 6: note = (2S,3S)-2-amino-3-(4-chloro-1H-indol-3-yl)butanoic acid
  SITE 8: note = d-N-methyl-Alanine
  SITE 10: note = l-Biphenylalanine-4-carboxylic acid
  SITE 12: note = l-2,4-diaminobutyric acid
  SITE 13: note = d-Alanine
  SITE 14: note = l-homoPhenylalanine
XWXGXXDAGXWXAX

SEQ ID NO: 143 - protein, 14 aa, synthetic construct
  SITE 1: note = l-Tyrosine O-ethyl acetamide
  SITE 3: note = l-phenylalanine-4-carboxylic acid
  SITE 5: note = (2S,4R)-4-aminopyrrolidine-2-carboxylic acid
  SITE 6: note = (2S,3S)-2-amino-3-(4-chloro-1H-indol-3-yl)butanoic acid
  SITE 8: note = d-N-methyl-Alanine
  SITE 10: note = l-Biphenylalanine-4-carboxylic acid
  SITE 12: note = l-2,4-diaminobutyric acid
  SITE 13: note = d-Alanine
  SITE 14: note = l-homoTyrosine
XWXGXXDAGXWXAX

SEQ ID NO: 144 - protein, 14 aa, synthetic construct
  SITE 1: note = l-Tyrosine O-ethyl acetamide
  SITE 3: note = l-phenylalanine-4-carboxylic acid
  SITE 5: note = (2S,4R)-4-aminopyrrolidine-2-carboxylic acid
  SITE 6: note = (2S,3S)-2-amino-3-(4-chloro-1H-indol-3-yl)butanoic acid
  SITE 8: note = d-N-methyl-Alanine
  SITE 10: note = l-Biphenylalanine-4-carboxylic acid
  SITE 12: note = l-2,3-diaminopropionic acid
  SITE 13: note = d-Alanine
  SITE 14: note = l-homoPhenylalanine
XWXGXXDAGXWXAX

SEQ ID NO: 145 - protein, 14 aa, synthetic construct
  SITE 1: note = l-Tyrosine O-ethyl acetamide
  SITE 3: note = l-phenylalanine-4-carboxylic acid
  SITE 5: note = (2S,4R)-4-aminopyrrolidine-2-carboxylic acid
  SITE 6: note = (2S,3S)-2-amino-3-(4-chloro-1H-indol-3-yl)butanoic acid
  SITE 8: note = d-N-methyl-Alanine
  SITE 10: note = l-Biphenylalanine-4-carboxylic acid
  SITE 12: note = l-2,3-diaminopropionic acid
  SITE 13: note = d-Alanine
  SITE 14: note = l-homoTyrosine
XWXGXXDAGXWXAX

SEQ ID NO: 146 - protein, 14 aa, synthetic construct
  SITE 1: note = l-Tyrosine O-ethyl acetamide
  SITE 3: note = l-phenylalanine-4-carboxylic acid
  SITE 5: note = (2S,4R)-4-aminopyrrolidine-2-carboxylic acid
  SITE 6: note = (2S,3S)-2-amino-3-(4-chloro-1H-indol-3-yl)butanoic acid
  SITE 8: note = d-N-methyl-Alanine
  SITE 10: note = l-Biphenylalanine-4-carboxylic acid
  SITE 12: note = (S)-2-amino-3-(dimethylamino)propanoic acid
  SITE 13: note = d-Alanine
  SITE 14: note = l-homoTyrosine
XWXGXXDAGXWXAX

SEQ ID NO: 147 - protein, 14 aa, synthetic construct
  SITE 1: note = l-Tyrosine O-ethyl acetamide
  SITE 3: note = l-phenylalanine-4-carboxylic acid
  SITE 5: note = (2S,4R)-4-aminopyrrolidine-2-carboxylic acid
  SITE 6: note = (2S,3S)-2-amino-3-(4-chloro-1H-indol-3-yl)butanoic acid
  SITE 8: note = d-N-methyl-Alanine
  SITE 10: note = l-Biphenylalanine-4-carboxylic acid
  SITE 12: note = (S)-2-amino-4-methoxybutanoic acid
  SITE 13: note = d-Alanine
  SITE 14: note = l-homoTyrosine
XWXGXXDAGXWXAX

SEQ ID NO: 148 - protein, 14 aa, synthetic construct
  SITE 1: note = l-Tyrosine O-ethyl acetamide
  SITE 3: note = l-phenylalanine-4-carboxylic acid
  SITE 5: note = (2S,4R)-4-aminopyrrolidine-2-carboxylic acid
  SITE 6: note = (2S,3S)-2-amino-3-(4-chloro-1H-indol-3-yl)butanoic acid
  SITE 8: note = d-N-methyl-Alanine
  SITE 10: note = l-Biphenylalanine-4-carboxylic acid
  SITE 13: note = d-Alanine
  SITE 14: note = l-homoTyrosine
XWXGXXDAGXWLAX

SEQ ID NO: 149 - protein, 14 aa, synthetic construct
  SITE 1: note = l-Tyrosine O-ethyl acetamide
  SITE 3: note = l-phenylalanine-4-carboxylic acid
  SITE 5: note = (2S,4R)-4-aminopyrrolidine-2-carboxylic acid
  SITE 6: note = (2S,3S)-2-amino-3-(4-chloro-1H-indol-3-yl)butanoic acid
  SITE 8: note = d-N-methyl-Alanine
  SITE 10: note = l-Biphenylalanine-4-carboxylic acid
  SITE 13: note = d-2,4-diaminobutyric acid
  SITE 14: note = l-homoTyrosine
XWXGXXDAGXWLXX

SEQ ID NO: 150 - protein, 14 aa, synthetic construct
  SITE 1: note = l-Tyrosine O-ethyl acetamide
  SITE 3: note = l-phenylalanine-4-carboxylic acid
  SITE 5: note = (2S,4R)-4-aminopyrrolidine-2-carboxylic acid
  SITE 6: note = (2S,3S)-2-amino-3-(4-chloro-1H-indol-3-yl)butanoic acid
  SITE 8: note = d-N-methyl-Alanine
  SITE 10: note = l-Biphenylalanine-4-carboxylic acid
  SITE 13: note = d-Alanine
  SITE 14: note = l-homoPhenylalanine
XWXGXXDAGXWSAX

SEQ ID NO: 151 - protein, 14 aa, synthetic construct
  SITE 1: note = l-Tyrosine O-ethyl acetamide
  SITE 3: note = l-phenylalanine-4-carboxylic acid
  SITE 5: note = (2S,4R)-4-aminopyrrolidine-2-carboxylic acid
  SITE 6: note = (2S,3S)-2-amino-3-(4-chloro-1H-indol-3-yl)butanoic acid
  SITE 8: note = d-N-methyl-Alanine
  SITE 10: note = l-Biphenylalanine-4-carboxylic acid
  SITE 13: note = d-Alanine
  SITE 14: note = l-homoTyrosine
XWXGXXDAGXWSAX

SEQ ID NO: 152 - protein, 14 aa, synthetic construct
  SITE 1: note = l-Tyrosine O-ethyl acetamide
  SITE 3: note = l-phenylalanine-4-carboxylic acid
  SITE 5: note = (2S,4R)-4-aminopyrrolidine-2-carboxylic acid
  SITE 6: note = (2S,3S)-2-amino-3-(4-chloro-1H-indol-3-yl)butanoic acid
  SITE 8: note = d-N-methyl-Alanine
  SITE 10: note = l-Biphenylalanine-4-carboxylic acid
  SITE 12: note = O-methyl-l-serine
  SITE 13: note = d-Alanine
  SITE 14: note = l-homoPhenylalanine
XWXGXXDAGXWSAX

SEQ ID NO: 153 - protein, 14 aa, synthetic construct
  SITE 1: note = l-Tyrosine O-ethyl acetamide
  SITE 3: note = l-phenylalanine-4-carboxylic acid
  SITE 5: note = (2S,4R)-4-aminopyrrolidine-2-carboxylic acid
  SITE 6: note = (2S,3S)-2-amino-3-(4-chloro-1H-indol-3-yl)butanoic acid
  SITE 8: note = d-N-methyl-Alanine
  SITE 10: note = l-Biphenylalanine-4-carboxylic acid
  SITE 12: note = O-methyl-l-serine
  SITE 13: note = d-Alanine
  SITE 14: note = l-homoTyrosine
XWXGXXDAGXWSAX

SEQ ID NO: 154 - protein, 14 aa, synthetic construct
  SITE 1: note = l-Tyrosine O-ethyl acetamide
  SITE 3: note = l-phenylalanine-4-carboxylic acid
  SITE 5: note = (2S,4R)-4-aminopyrrolidine-2-carboxylic acid
  SITE 6: note = (2S,3S)-2-amino-3-(4-fluoro-1H-indol-3-yl)butanoic acid
  SITE 8: note = d-N-methyl-Alanine
  SITE 10: note = l-Biphenylalanine-4-carboxylic acid
  SITE 11: note = 3-(1-Naphthyl)-l-alanine
  SITE 12: note = l-2,4-diaminobutyric acid
  SITE 13: note = d-Alanine
  SITE 14: note = l-homoTyrosine
XWXGXXDAGXXXAX

SEQ ID NO: 155 - protein, 14 aa, synthetic construct
  SITE 1: note = l-Tyrosine O-ethyl acetamide
  SITE 3: note = l-phenylalanine-4-carboxylic acid
  SITE 5: note = (2S,4R)-4-aminopyrrolidine-2-carboxylic acid
  SITE 6: note = (2S,3S)-2-amino-3-(4-fluoro-1H-indol-3-yl)butanoic acid
  SITE 8: note = d-N-methyl-Alanine
  SITE 10: note = l-Biphenylalanine-4-carboxylic acid
  SITE 11: note = 3-(1-Naphthyl)-l-alanine
  SITE 13: note = d-Alanine
  SITE 14: note = l-homoTyrosine
XWXGXXDAGXXSAX

SEQ ID NO: 156 - protein, 14 aa, synthetic construct
  SITE 1: note = l-Tyrosine O-ethyl acetamide
  SITE 3: note = l-phenylalanine-4-carboxylic acid
  SITE 5: note = (2S,4R)-4-aminopyrrolidine-2-carboxylic acid
  SITE 6: note = (2S,3S)-2-amino-3-(4-fluoro-1H-indol-3-yl)butanoic acid
  SITE 8: note = d-N-methyl-Alanine
  SITE 10: note = l-Biphenylalanine-4-carboxylic acid
  SITE 11: note = 4-Pyridylalanine
  SITE 13: note = d-Alanine
  SITE 14: note = l-homoTyrosine
XWXGXXDAGXXLAX

SEQ ID NO: 157 - protein, 14 aa, synthetic construct
  SITE 1: note = l-Tyrosine O-ethyl acetamide
  SITE 3: note = l-phenylalanine-4-carboxylic acid
  SITE 5: note = (2S,4R)-4-aminopyrrolidine-2-carboxylic acid
  SITE 6: note = (2S,3S)-2-amino-3-(4-fluoro-1H-indol-3-yl)butanoic acid
  SITE 8: note = d-N-methyl-Alanine
  SITE 10: note = l-Biphenylalanine-4-carboxylic acid
  SITE 11: note = 4-Pyridylalanine
  SITE 12: note = l-Norvaline
  SITE 13: note = d-Alanine
  SITE 14: note = l-homoTyrosine
XWXGXXDAGXXXAX

SEQ ID NO: 158 - protein, 14 aa, synthetic construct
  SITE 1: note = l-Tyrosine O-ethyl acetamide
  SITE 3: note = l-phenylalanine-4-carboxylic acid
  SITE 5: note = (2S,4R)-4-aminopyrrolidine-2-carboxylic acid
  SITE 6: note = (2S,3S)-2-amino-3-(4-fluoro-1H-indol-3-yl)butanoic acid
  SITE 8: note = d-N-methyl-Alanine
  SITE 10: note = l-Biphenylalanine-4-carboxylic acid
  SITE 13: note = d-Alanine
  SITE 14: note = (S)-2-amino-4-(5-cyanopyridin-3-yl)butanoic acid
XWXGXXDAGXKLAX

SEQ ID NO: 159 - protein, 14 aa, synthetic construct
  SITE 1: note = l-Tyrosine O-ethyl acetamide
  SITE 3: note = l-phenylalanine-4-carboxylic acid
  SITE 5: note = (2S,4R)-4-aminopyrrolidine-2-carboxylic acid
  SITE 6: note = (2S,3S)-2-amino-3-(4-fluoro-1H-indol-3-yl)butanoic acid
  SITE 8: note = d-N-methyl-Alanine
  SITE 10: note = l-Biphenylalanine-4-carboxylic acid
  SITE 13: note = d-Alanine
  SITE 14: note = l-homoTyrosine
XWXGXXDAGXKLAX

SEQ ID NO: 160 - protein, 14 aa, synthetic construct
  SITE 1: note = l-Tyrosine O-ethyl acetamide
  SITE 3: note = l-phenylalanine-4-carboxylic acid
  SITE 5: note = (2S,4R)-4-aminopyrrolidine-2-carboxylic acid
  SITE 6: note = (2S,3S)-2-amino-3-(4-fluoro-1H-indol-3-yl)butanoic acid
  SITE 8: note = d-N-methyl-Alanine
  SITE 10: note = l-Biphenylalanine-4-carboxylic acid
  SITE 13: note = d-2,4-diaminobutyric acid
  SITE 14: note = l-homoTyrosine
XWXGXXDAGXKLXX

SEQ ID NO: 161 - protein, 14 aa, synthetic construct
  SITE 1: note = l-Tyrosine O-ethyl acetamide
  SITE 3: note = l-phenylalanine-4-carboxylic acid
  SITE 5: note = (2S,4R)-4-aminopyrrolidine-2-carboxylic acid
  SITE 6: note = (2S,3S)-2-amino-3-(4-fluoro-1H-indol-3-yl)butanoic acid
  SITE 8: note = d-N-methyl-Alanine
  SITE 10: note = l-Biphenylalanine-4-carboxylic acid
  SITE 13: note = d-Serine
  SITE 14: note = l-homoTyrosine
XWXGXXDAGXKLSX

SEQ ID NO: 162 - protein, 14 aa, synthetic construct
  SITE 1: note = l-Tyrosine O-ethyl acetamide
  SITE 3: note = l-phenylalanine-4-carboxylic acid
  SITE 5: note = (2S,4R)-4-aminopyrrolidine-2-carboxylic acid
  SITE 6: note = (2S,3S)-2-amino-3-(4-fluoro-1H-indol-3-yl)butanoic acid
  SITE 8: note = d-N-methyl-Alanine
  SITE 10: note = l-Biphenylalanine-4-carboxylic acid
  SITE 12: note = (S)-2-amino-4-morpholinobutanoic acid
  SITE 13: note = d-Alanine
XWXGXXDAGXWXAG

SEQ ID NO: 163 - protein, 14 aa, synthetic construct
  SITE 1: note = l-Tyrosine O-ethyl acetamide
  SITE 3: note = l-phenylalanine-4-carboxylic acid
  SITE 5: note = (2S,4R)-4-aminopyrrolidine-2-carboxylic acid
  SITE 6: note = (2S,3S)-2-amino-3-(4-fluoro-1H-indol-3-yl)butanoic acid
  SITE 8: note = d-N-methyl-Alanine
  SITE 10: note = l-Biphenylalanine-4-carboxylic acid
  SITE 12: note = l-2,4-diaminobutyric acid
  SITE 13: note = d-Alanine
  SITE 14: note = l-homoPhenylalanine
XWXGXXDAGXWXAX

SEQ ID NO: 164 - protein, 14 aa, synthetic construct
  SITE 1: note = l-Tyrosine O-ethyl acetamide
  SITE 3: note = l-phenylalanine-4-carboxylic acid
  SITE 5: note = (2S,4R)-4-aminopyrrolidine-2-carboxylic acid
  SITE 6: note = (2S,3S)-2-amino-3-(4-fluoro-1H-indol-3-yl)butanoic acid
  SITE 8: note = d-N-methyl-Alanine
  SITE 10: note = l-Biphenylalanine-4-carboxylic acid
  SITE 13: note = d-Alanine
  SITE 14: note = (S)-2-amino-3-(6-(2-aminoethoxy)pyridin-3-yl)propanoic acid
XWXGXXDAGXWLAX

SEQ ID NO: 165 - protein, 14 aa, synthetic construct
  SITE 1: note = l-Tyrosine O-ethyl acetamide
  SITE 3: note = l-phenylalanine-4-carboxylic acid
  SITE 5: note = (2S,4R)-4-aminopyrrolidine-2-carboxylic acid
  SITE 6: note = (2S,3S)-2-amino-3-(4-fluoro-1H-indol-3-yl)butanoic acid
  SITE 8: note = d-N-methyl-Alanine
  SITE 10: note = l-Biphenylalanine-4-carboxylic acid
  SITE 13: note = d-Alanine
  SITE 14: note = (S)-2-amino-3-(piperidin-4-yl)propanoic acid
XWXGXXDAGXWLAX

SEQ ID NO: 166 - protein, 14 aa, synthetic construct
  SITE 1: note = l-Tyrosine O-ethyl acetamide
  SITE 3: note = l-phenylalanine-4-carboxylic acid
  SITE 5: note = (2S,4R)-4-aminopyrrolidine-2-carboxylic acid
  SITE 6: note = (2S,3S)-2-amino-3-(4-fluoro-1H-indol-3-yl)butanoic acid
  SITE 8: note = d-N-methyl-Alanine
  SITE 10: note = l-Biphenylalanine-4-carboxylic acid
  SITE 13: note = d-Alanine
  SITE 14: note = l-homoPhenylalanine
XWXGXXDAGXWLAX

SEQ ID NO: 167 - protein, 14 aa, synthetic construct
  SITE 1: note = l-Tyrosine O-ethyl acetamide
  SITE 3: note = l-phenylalanine-4-carboxylic acid
  SITE 5: note = (2S,4R)-4-aminopyrrolidine-2-carboxylic acid
  SITE 6: note = (2S,3S)-2-amino-3-(4-fluoro-1H-indol-3-yl)butanoic acid
  SITE 8: note = d-N-methyl-Alanine
  SITE 10: note = l-Biphenylalanine-4-carboxylic acid
  SITE 13: note = d-Alanine
  SITE 14: note = l-homoTyrosine
XWXGXXDAGXWLAX

SEQ ID NO: 168 - protein, 14 aa, synthetic construct
  SITE 1: note = l-Tyrosine O-ethyl acetamide
  SITE 3: note = l-phenylalanine-4-carboxylic acid
  SITE 5: note = (2S,4R)-4-aminopyrrolidine-2-carboxylic acid
  SITE 6: note = (2S,3S)-2-amino-3-(4-fluoro-1H-indol-3-yl)butanoic acid
  SITE 8: note = d-N-methyl-Alanine
  SITE 10: note = l-Biphenylalanine-4-carboxylic acid
  SITE 13: note = d-2,4-diaminobutyric acid
  SITE 14: note = l-homoTyrosine
XWXGXXDAGXWLXX

SEQ ID NO: 169 - protein, 14 aa, synthetic construct
  SITE 1: note = l-Tyrosine O-ethyl acetamide
  SITE 3: note = l-phenylalanine-4-carboxylic acid
  SITE 5: note = (2S,4R)-4-aminopyrrolidine-2-carboxylic acid
  SITE 6: note = (2S,3S)-2-amino-3-(4-fluoro-1H-indol-3-yl)butanoic acid
  SITE 8: note = d-N-methyl-Alanine
  SITE 10: note = l-Biphenylalanine-4-carboxylic acid
  SITE 13: note = d-Lysine
  SITE 14: note = l-homoTyrosine
XWXGXXDAGXWLKX

SEQ ID NO: 170 - protein, 14 aa, synthetic construct
  SITE 1: note = l-Tyrosine O-ethyl acetamide
  SITE 3: note = l-phenylalanine-4-carboxylic acid
  SITE 5: note = (2S,4R)-4-aminopyrrolidine-2-carboxylic acid
  SITE 6: note = (2S,3S)-2-amino-3-(4-fluoro-1H-indol-3-yl)butanoic acid
  SITE 8: note = d-N-methyl-Alanine
  SITE 10: note = l-Biphenylalanine-4-carboxylic acid
  SITE 13: note = d-Ornithine
  SITE 14: note = l-homoTyrosine
XWXGXXDAGXWLXX

SEQ ID NO: 171 - protein, 14 aa, synthetic construct
  SITE 1: note = l-Tyrosine O-ethyl acetamide
  SITE 3: note = l-phenylalanine-4-carboxylic acid
  SITE 5: note = (2S,4R)-4-aminopyrrolidine-2-carboxylic acid
  SITE 6: note = (2S,3S)-2-amino-3-(4-fluoro-1H-indol-3-yl)butanoic acid
  SITE 8: note = d-N-methyl-Alanine
  SITE 10: note = l-Biphenylalanine-4-carboxylic acid
  SITE 13: note = d-Serine
  SITE 14: note = l-homoTyrosine
XWXGXXDAGXWLSX

SEQ ID NO: 172 - protein, 14 aa, synthetic construct
  SITE 1: note = l-Tyrosine O-ethyl acetamide
  SITE 3: note = l-phenylalanine-4-carboxylic acid
  SITE 5: note = (2S,4R)-4-aminopyrrolidine-2-carboxylic acid
  SITE 6: note = (2S,3S)-2-amino-3-(4-fluoro-1H-indol-3-yl)butanoic acid
  SITE 8: note = d-N-methyl-Alanine
  SITE 10: note = l-Biphenylalanine-4-carboxylic acid
  SITE 13: note = d-Alanine
  SITE 14: note = l-homoTyrosine
XWXGXXDAGXWSAX

SEQ ID NO: 173 - protein, 14 aa, synthetic construct
  SITE 1: note = l-Tyrosine O-ethyl acetamide
  SITE 3: note = l-phenylalanine-4-carboxylic acid
  SITE 5: note = (2S,4R)-4-aminopyrrolidine-2-carboxylic acid
  SITE 6: note = (2S,3S)-2-amino-3-(4-fluoro-1H-indol-3-yl)butanoic acid
  SITE 8: note = d-N-methyl-Alanine
  SITE 10: note = l-Biphenylalanine-4-carboxylic acid
  SITE 13: note = d-Alanine
  SITE 14: note = l-Tyrosine O-ethyl acetamide
XWXGXXDAGXWSAX

SEQ ID NO: 174 - protein, 14 aa, synthetic construct
  SITE 1: note = (S)-3-(6-(4-acetylpiperazin-1-yl)pyridin-3-yl)-2-aminopropanoic acid
  SITE 3: note = l-phenylalanine-4-carboxylic acid
  SITE 5: note = (2S,4R)-4-aminopyrrolidine-2-carboxylic acid
  SITE 6: note = (2S,3S)-2-amino-3-(naphthalen-1-yl)butanoic acid
  SITE 8: note = d-N-methyl-Alanine
  SITE 10: note = l-Biphenylalanine-4-carboxylic acid
  SITE 11: note = l-2,4-diaminobutyric acid
  SITE 13: note = d-Alanine
  SITE 14: note = (S)-2-amino-4-cyclohexylbutanoic acid
XWXGXXDAGXXLAX

SEQ ID NO: 175 - protein, 14 aa, synthetic construct
  SITE 1: note = (S)-3-(6-(4-acetylpiperazin-1-yl)pyridin-3-yl)-2-aminopropanoic acid
  SITE 3: note = l-phenylalanine-4-carboxylic acid
  SITE 5: note = (2S,4R)-4-aminopyrrolidine-2-carboxylic acid
  SITE 6: note = (2S,3S)-2-amino-3-(naphthalen-1-yl)butanoic acid
  SITE 8: note = d-N-methyl-Alanine
  SITE 10: note = l-Biphenylalanine-4-carboxylic acid
  SITE 11: note = l-2,3-diaminopropionic acid
  SITE 13: note = d-Alanine
  SITE 14: note = (S)-2-amino-4-cyclohexylbutanoic acid
XWXGXXDAGXXLAX

SEQ ID NO: 176 - protein, 14 aa, synthetic construct
  SITE 1: note = (S)-3-(6-(4-acetylpiperazin-1-yl)pyridin-3-yl)-2-aminopropanoic acid
  SITE 3: note = l-phenylalanine-4-carboxylic acid
  SITE 5: note = (2S,4R)-4-aminopyrrolidine-2-carboxylic acid
  SITE 6: note = (2S,3S)-2-amino-3-(naphthalen-1-yl)butanoic acid
  SITE 8: note = d-N-methyl-Alanine
  SITE 10: note = l-Biphenylalanine-4-carboxylic acid
  SITE 11: note = l-homoGlutamine
  SITE 13: note = d-Alanine
  SITE 14: note = (S)-2-amino-4-(5-cyanopyridin-3-yl)butanoic acid
XWXGXXDAGXXLAX

SEQ ID NO: 177 - protein, 14 aa, synthetic construct
  SITE 1: note = (S)-3-(6-(4-acetylpiperazin-1-yl)pyridin-3-yl)-2-aminopropanoic acid
  SITE 3: note = l-phenylalanine-4-carboxylic acid
  SITE 5: note = (2S,4R)-4-aminopyrrolidine-2-carboxylic acid
  SITE 6: note = (2S,3S)-2-amino-3-(naphthalen-1-yl)butanoic acid
  SITE 8: note = d-N-methyl-Alanine
  SITE 10: note = l-Biphenylalanine-4-carboxylic acid
  SITE 13: note = d-Alanine
  SITE 14: note = (S)-2-amino-4-cyclohexylbutanoic acid
XWXGXXDAGXKLAX

SEQ ID NO: 178 - protein, 14 aa, synthetic construct
  SITE 1: note = (S)-3-(6-(4-acetylpiperazin-1-yl)pyridin-3-yl)-2-aminopropanoic acid
  SITE 3: note = l-phenylalanine-4-carboxylic acid
  SITE 5: note = (2S,4R)-4-aminopyrrolidine-2-carboxylic acid
  SITE 6: note = (2S,3S)-2-amino-3-(naphthalen-1-yl)butanoic acid
  SITE 8: note = d-N-methyl-Alanine
  SITE 10: note = l-Biphenylalanine-4-carboxylic acid
  SITE 13: note = d-Leucine
  SITE 14: note = (S)-2-amino-4-(5-cyanopyridin-3-yl)butanoic acid
XWXGXXDAGXKLLX

SEQ ID NO: 179 - protein, 14 aa, synthetic construct
  SITE 1: note = (S)-3-(6-(4-acetylpiperazin-1-yl)pyridin-3-yl)-2-aminopropanoic acid
  SITE 3: note = l-phenylalanine-4-carboxylic acid
  SITE 5: note = (2S,4R)-4-aminopyrrolidine-2-carboxylic acid
  SITE 6: note = (2S,3S)-2-amino-3-(naphthalen-1-yl)butanoic acid
  SITE 8: note = d-N-methyl-Alanine
  SITE 10: note = l-Biphenylalanine-4-carboxylic acid
  SITE 13: note = d-Norleucine
  SITE 14: note = (S)-2-amino-4-(5-cyanopyridin-3-yl)butanoic acid
XWXGXXDAGXKLXX

SEQ ID NO: 180 - protein, 14 aa, synthetic construct
  SITE 1: note = (S)-3-(6-(4-acetylpiperazin-1-yl)pyridin-3-yl)-2-aminopropanoic acid
  SITE 3: note = l-phenylalanine-4-carboxylic acid
  SITE 5: note = (2S,4R)-4-aminopyrrolidine-2-carboxylic acid
  SITE 6: note = (2S,3S)-2-amino-3-(naphthalen-1-yl)butanoic acid
  SITE 8: note = d-N-methyl-Alanine
  SITE 10: note = l-Biphenylalanine-4-carboxylic acid
  SITE 13: note = d-Norvaline
  SITE 14: note = (S)-2-amino-4-(5-cyanopyridin-3-yl)butanoic acid
XWXGXXDAGXKLXX

SEQ ID NO: 181 - protein, 14 aa, synthetic construct
  SITE 1: note = (S)-3-(6-(4-acetylpiperazin-1-yl)pyridin-3-yl)-2-aminopropanoic acid
  SITE 3: note = l-phenylalanine-4-carboxylic acid
  SITE 5: note = (2S,4R)-4-aminopyrrolidine-2-carboxylic acid
  SITE 6: note = (2S,3S)-2-amino-3-(naphthalen-1-yl)butanoic acid
  SITE 8: note = d-N-methyl-Alanine
  SITE 10: note = l-Biphenylalanine-4-carboxylic acid
  SITE 12: note = (S)-2-amino-4,4-dimethylpentanoic acid
  SITE 13: note = d-Alanine
  SITE 14: note = (S)-2-amino-4-(5-cyanopyridin-3-yl)butanoic acid
XWXGXXDAGXKXAX

SEQ ID NO: 182 - protein, 14 aa, synthetic construct
  SITE 1: note = (S)-3-(6-(4-acetylpiperazin-1-yl)pyridin-3-yl)-2-aminopropanoic acid
  SITE 3: note = l-phenylalanine-4-carboxylic acid
  SITE 5: note = (2S,4R)-4-aminopyrrolidine-2-carboxylic acid
  SITE 6: note = (2S,3S)-2-amino-3-(naphthalen-1-yl)butanoic acid
  SITE 8: note = d-N-methyl-Alanine
  SITE 10: note = l-Biphenylalanine-4-carboxylic acid
  SITE 11: note = l-Ornithine
  SITE 13: note = d-Alanine
  SITE 14: note = (S)-2-amino-4-cyclohexylbutanoic acid
XWXGXXDAGXXLAX

SEQ ID NO: 183 - protein, 14 aa, synthetic construct
  SITE 1: note = (S)-3-(6-(4-acetylpiperazin-1-yl)pyridin-3-yl)-2-aminopropanoic acid
  SITE 3: note = l-phenylalanine-4-carboxylic acid
  SITE 5: note = (2S,4R)-4-aminopyrrolidine-2-carboxylic acid
  SITE 6: note = (2S,3S)-2-amino-3-(naphthalen-1-yl)butanoic acid
  SITE 8: note = d-N-methyl-Alanine
  SITE 10: note = l-Biphenylalanine-4-carboxylic acid
  SITE 13: note = d-Alanine
  SITE 14: note = (S)-2-amino-4-(5-cyanopyridin-3-yl)butanoic acid
XWXGXXDAGXQLAX

SEQ ID NO: 184 - protein, 14 aa, synthetic construct
  SITE 1: note = l-Biphenylalanine-4-carboxylic acid
  SITE 2: note = (S)-2-amino-3-(6-chloro-1H-indol-3-yl)propanoic acid
  SITE 3: note = l-phenylalanine-4-carboxylic acid
  SITE 5: note = (2S,4R)-4-aminopyrrolidine-2-carboxylic acid
  SITE 6: note = (2S,3S)-2-amino-3-(4-fluoro-1H-indol-3-yl)butanoic acid
  SITE 8: note = d-N-methyl-Alanine
  SITE 10: note = l-Biphenylalanine-4-carboxylic acid
  SITE 13: note = d-Alanine
  SITE 14: note = l-homoTyrosine
XXXGXXDAGXKLAX

SEQ ID NO: 185 - protein, 14 aa, synthetic construct
  SITE 1: note = l-Biphenylalanine-4-carboxylic acid
  SITE 2: note = (S)-2-amino-3-(7-fluoro-1H-indol-3-yl)propanoic acid
  SITE 3: note = l-phenylalanine-4-carboxylic acid
  SITE 5: note = (2S,4R)-4-aminopyrrolidine-2-carboxylic acid
  SITE 6: note = (2S,3S)-2-amino-3-(4-fluoro-1H-indol-3-yl)butanoic acid
  SITE 8: note = d-N-methyl-Alanine
  SITE 10: note = l-Biphenylalanine-4-carboxylic acid
  SITE 13: note = d-Alanine
  SITE 14: note = l-homoTyrosine
XXXGXXDAGXKLAX

SEQ ID NO: 186 - protein, 14 aa, synthetic construct
  SITE 1: note = l-Biphenylalanine-4-carboxylic acid
  SITE 2: note = (S)-2-amino-3-(7-methyl-1H-indol-3-yl)propanoic acid
  SITE 3: note = l-phenylalanine-4-carboxylic acid
  SITE 5: note = (2S,4R)-4-aminopyrrolidine-2-carboxylic acid
  SITE 6: note = (2S,3S)-2-amino-3-(4-fluoro-1H-indol-3-yl)butanoic acid
  SITE 8: note = d-N-methyl-Alanine
  SITE 10: note = l-Biphenylalanine-4-carboxylic acid
  SITE 13: note = d-Alanine
  SITE 14: note = l-homoTyrosine
XXXGXXDAGXKLAX

SEQ ID NO: 187 - protein, 14 aa, synthetic construct
  SITE 1: note = l-Biphenylalanine-4-carboxylic acid
  SITE 3: note = l-phenylalanine-4-carboxylic acid
  SITE 5: note = (2S,4R)-4-aminopyrrolidine-2-carboxylic acid
  SITE 6: note = (2S,3S)-2-amino-3-(4-fluoro-1H-indol-3-yl)butanoic acid
  SITE 8: note = d-N-methyl-Alanine
  SITE 10: note = l-Biphenylalanine-4-carboxylic acid
  SITE 13: note = (R)-6-acetamido-2-aminohexanoic acid
  SITE 14: note = l-homoTyrosine
XWXGXXDAGXKLKX

SEQ ID NO: 188 - protein, 14 aa, synthetic construct
  SITE 1: note = 3-[4-[(S)-2-amino-2-carboxyethyl]phenyl]bicyclo[1.1.1]pentane-1-carboxylic acid
  SITE 3: note = l-phenylalanine-4-carboxylic acid
  SITE 5: note = (2S,4R)-4-aminopyrrolidine-2-carboxylic acid
  SITE 6: note = (2S,3S)-2-amino-3-(naphthalen-1-yl)butanoic acid
  SITE 8: note = d-N-methyl-Alanine
  SITE 10: note = l-Biphenylalanine-4-carboxylic acid
  SITE 11: note = (S)-2-amino-3-(1H-indazol-1-yl)propanoic acid
  SITE 13: note = d-2,4-diaminobutyric acid
  SITE 14: note = (S)-2-amino-4-cyclohexylbutanoic acid
XWXGXXDAGXXGXX

SEQ ID NO: 189 - protein, 14 aa, synthetic construct
  SITE 1: note = 3-[4-[(S)-2-amino-2-carboxyethyl]phenyl]bicyclo[1.1.1]pentane-1-carboxylic acid
  SITE 3: note = l-phenylalanine-4-carboxylic acid
  SITE 5: note = (2S,4R)-4-aminopyrrolidine-2-carboxylic acid
  SITE 6: note = (2S,3S)-2-amino-3-(naphthalen-1-yl)butanoic acid
  SITE 8: note = d-N-methyl-Alanine
  SITE 10: note = l-Biphenylalanine-4-carboxylic acid
  SITE 11: note = (S)-2-amino-3-cyclohexylpropanoic acid
  SITE 13: note = d-2,4-diaminobutyric acid
  SITE 14: note = (S)-2-amino-4-cyclohexylbutanoic acid
XWXGXXDAGXXGXX

SEQ ID NO: 190 - protein, 14 aa, synthetic construct
  SITE 1: note = 3-[4-[(S)-2-amino-2-carboxyethyl]phenyl]bicyclo[1.1.1]pentane-1-carboxylic acid
  SITE 3: note = l-phenylalanine-4-carboxylic acid
  SITE 5: note = (2S,4R)-4-aminopyrrolidine-2-carboxylic acid
  SITE 6: note = (2S,3S)-2-amino-3-(naphthalen-1-yl)butanoic acid
  SITE 8: note = d-N-methyl-Alanine
  SITE 10: note = l-Biphenylalanine-4-carboxylic acid
  SITE 11: note = (S)-2-amino-3-cyclohexylpropanoic acid
  SITE 13: note = d-2,4-diaminobutyric acid
  SITE 14: note = l-homoTyrosine
XWXGXXDAGXXGXX

SEQ ID NO: 191 - protein, 14 aa, synthetic construct
  SITE 1: note = (1R,4s)-4-(4-((S)-2-amino-2-carboxyethyl)phenyl)cyclohexane-1-carboxylic acid
  SITE 3: note = l-phenylalanine-4-carboxylic acid
  SITE 5: note = (2S,4R)-4-aminopyrrolidine-2-carboxylic acid
  SITE 6: note = (2S,3S)-2-amino-3-(naphthalen-1-yl)butanoic acid
  SITE 8: note = d-N-methyl-Alanine
  SITE 10: note = l-Biphenylalanine-4-carboxylic acid
  SITE 11: note = 4-Pyridylalanine
  SITE 13: note = d-2,4-diaminobutyric acid
  SITE 14: note = (S)-2-amino-4-cyclohexylbutanoic acid
XWXGXXDAGXXGXX

SEQ ID NO: 192 - protein, 14 aa, synthetic construct
  SITE 1: note = (1S,4r)-4-(4-((S)-2-amino-2-carboxyethyl)phenyl)cyclohexane-1-carboxylic acid
  SITE 2: note = (S)-2-amino-3-(6-fluoro-1H-indol-3-yl)propanoic acid
  SITE 3: note = l-phenylalanine-4-carboxylic acid
  SITE 5: note = (2S,4R)-4-aminopyrrolidine-2-carboxylic acid
  SITE 6: note = (2S,3S)-2-amino-3-(naphthalen-1-yl)butanoic acid
  SITE 8: note = d-N-methyl-Alanine
  SITE 10: note = l-Biphenylalanine-4-carboxylic acid
  SITE 11: note = 4-Pyridylalanine
  SITE 13: note = d-2,4-diaminobutyric acid
  SITE 14: note = (S)-2-amino-4-cyclohexylbutanoic acid
XXXGXXDAGXXGXX

SEQ ID NO: 193 - protein, 14 aa, synthetic construct
  SITE 1: note = (1S,4r)-4-(4-((S)-2-amino-2-carboxyethyl)phenyl)cyclohexane-1-carboxylic acid
  SITE 2: note = (S)-2-amino-3-(6-fluoro-1H-indol-3-yl)propanoic acid
  SITE 3: note = l-phenylalanine-4-carboxylic acid
  SITE 5: note = (2S,4R)-4-aminopyrrolidine-2-carboxylic acid
  SITE 6: note = (2S,3S)-2-amino-3-(naphthalen-1-yl)butanoic acid
  SITE 8: note = d-N-methyl-Alanine
  SITE 10: note = l-Biphenylalanine-4-carboxylic acid
  SITE 11: note = 4-Pyridylalanine
  SITE 13: note = d-2,4-diaminobutyric acid
  SITE 14: note = (S)-2-amino-4-cyclohexylbutanoic acid
XXXGXXDAGXXSXX

SEQ ID NO: 194 - protein, 14 aa, synthetic construct
  SITE 1: note = (1S,4r)-4-(4-((S)-2-amino-2-carboxyethyl)phenyl)cyclohexane-1-carboxylic acid
  SITE 2: note = (S)-2-amino-3-(6-fluoro-1H-indol-3-yl)propanoic acid
  SITE 3: note = l-phenylalanine-4-carboxylic acid
  SITE 5: note = (2S,4R)-4-aminopyrrolidine-2-carboxylic acid
  SITE 6: note = (2S,3S)-2-amino-3-(naphthalen-1-yl)butanoic acid
  SITE 8: note = d-N-methyl-Alanine
  SITE 10: note = l-Biphenylalanine-4-carboxylic acid
  SITE 11: note = 4-Pyridylalanine
  SITE 13: note = [(R)-3-amino-3-carboxypropyl]-trimethylazanium
  SITE 14: note = (S)-2-amino-4-cyclohexylbutanoic acid
XXXGXXDAGXXSXX

SEQ ID NO: 195 - protein, 14 aa, synthetic construct
  SITE 1: note = (1S,4r)-4-(4-((S)-2-amino-2-carboxyethyl)phenyl)cyclohexane-1-carboxylic acid
  SITE 3: note = l-phenylalanine-4-carboxylic acid
  SITE 5: note = (2S,4R)-4-aminopyrrolidine-2-carboxylic acid
  SITE 6: note = (2S,3S)-2-amino-3-(naphthalen-1-yl)butanoic acid
  SITE 8: note = d-N-methyl-Alanine
  SITE 10: note = l-Biphenylalanine-4-carboxylic acid
  SITE 11: note = 4-Pyridylalanine
  SITE 13: note = d-2,4-diaminobutyric acid
  SITE 14: note = (S)-2-amino-2-methylhexanoic acid
XWXGXXDAGXXGXX

SEQ ID NO: 196 - protein, 14 aa, synthetic construct
  SITE 1: note = (1S,4r)-4-(4-((S)-2-amino-2-carboxyethyl)phenyl)cyclohexane-1-carboxylic acid
  SITE 3: note = l-phenylalanine-4-carboxylic acid
  SITE 5: note = (2S,4R)-4-aminopyrrolidine-2-carboxylic acid
  SITE 6: note = (2S,3S)-2-amino-3-(naphthalen-1-yl)butanoic acid
  SITE 8: note = d-N-methyl-Alanine
  SITE 10: note = l-Biphenylalanine-4-carboxylic acid
  SITE 11: note = 4-Pyridylalanine
  SITE 13: note = d-2,4-diaminobutyric acid
  SITE 14: note = (S)-2-amino-4-cyclohexylbutanoic acid
XWXGXXDAGXXGXX

SEQ ID NO: 197 - protein, 14 aa, synthetic construct
  SITE 1: note = (1S,4r)-4-(4-((S)-2-amino-2-carboxyethyl)phenyl)cyclohexane-1-carboxylic acid
  SITE 3: note = l-phenylalanine-4-carboxylic acid
  SITE 5: note = (2S,4R)-4-aminopyrrolidine-2-carboxylic acid
  SITE 6: note = (2S,3S)-2-amino-3-(naphthalen-1-yl)butanoic acid
  SITE 8: note = d-N-methyl-Alanine
  SITE 10: note = l-Biphenylalanine-4-carboxylic acid
  SITE 11: note = 4-Pyridylalanine
  SITE 13: note = d-2,4-diaminobutyric acid
  SITE 14: note = l-Norleucine
XWXGXXDAGXXGXX

SEQ ID NO: 198 - protein, 14 aa, synthetic construct
  SITE 1: note = (S)-2-amino-3-(4-(4-acetylpiperazin-1-yl)phenyl)propanoic acid
  SITE 3: note = l-phenylalanine-4-carboxylic acid
  SITE 5: note = (2S,4R)-4-aminopyrrolidine-2-carboxylic acid
  SITE 6: note = (2S,3S)-2-amino-3-(naphthalen-1-yl)butanoic acid
  SITE 8: note = d-N-methyl-Alanine
  SITE 10: note = l-Biphenylalanine-4-carboxylic acid
  SITE 11: note = (S)-2-amino-3-(indolin-1-yl)propanoic acid
  SITE 13: note = d-2,4-diaminobutyric acid
  SITE 14: note = l-homoTyrosine
XWXGXXDAGXXGXX

SEQ ID NO: 199 - protein, 14 aa, synthetic construct
  SITE 1: note = (S)-2-amino-3-(4-(4-acetylpiperazin-1-yl)phenyl)propanoic acid
  SITE 3: note = l-phenylalanine-4-carboxylic acid
  SITE 5: note = (2S,4R)-4-aminopyrrolidine-2-carboxylic acid
  SITE 6: note = (2S,3S)-2-amino-3-(naphthalen-1-yl)butanoic acid
  SITE 8: note = d-N-methyl-Alanine
  SITE 10: note = l-Biphenylalanine-4-carboxylic acid
  SITE 11: note = 4-Pyridylalanine
  SITE 13: note = (R)-2,4-diamino-2-methylbutanal
  SITE 14: note = (S)-2-amino-4-cyclohexylbutanoic acid
XWXGXXDAGXXGXX

SEQ ID NO: 200 - protein, 14 aa, synthetic construct
  SITE 1: note = (S)-2-amino-3-(4-(4-acetylpiperazin-1-yl)phenyl)propanoic acid
  SITE 3: note = l-phenylalanine-4-carboxylic acid
  SITE 5: note = (2S,4R)-4-aminopyrrolidine-2-carboxylic acid
  SITE 6: note = (2S,3S)-2-amino-3-(naphthalen-1-yl)butanoic acid
  SITE 8: note = d-N-methyl-Alanine
  SITE 10: note = l-Biphenylalanine-4-carboxylic acid
  SITE 11: note = 4-Pyridylalanine
  SITE 13: note = d-2,4-diaminobutyric acid
  SITE 14: note = (S)-2-amino-2-methylhexanoic acid
XWXGXXDAGXXGXX

SEQ ID NO: 201 - protein, 14 aa, synthetic construct
  SITE 1: note = (S)-2-amino-3-(4-(4-acetylpiperazin-1-yl)phenyl)propanoic acid
  SITE 3: note = l-phenylalanine-4-carboxylic acid
  SITE 5: note = (2S,4R)-4-aminopyrrolidine-2-carboxylic acid
  SITE 6: note = (2S,3S)-2-amino-3-(naphthalen-1-yl)butanoic acid
  SITE 8: note = d-N-methyl-Alanine
  SITE 10: note = l-Biphenylalanine-4-carboxylic acid
  SITE 11: note = 4-Pyridylalanine
  SITE 13: note = d-2,4-diaminobutyric acid
  SITE 14: note = (S)-2-amino-4-cyclohexylbutanoic acid
XWXGXXDAGXXGXX

SEQ ID NO: 202 - protein, 14 aa, synthetic construct
  SITE 1: note = (S)-2-amino-3-(4-(4-acetylpiperazin-1-yl)phenyl)propanoic acid
  SITE 3: note = l-phenylalanine-4-carboxylic acid
  SITE 5: note = (2S,4R)-4-aminopyrrolidine-2-carboxylic acid
  SITE 6: note = (2S,3S)-2-amino-3-(naphthalen-1-yl)butanoic acid
  SITE 8: note = d-N-methyl-Alanine
  SITE 10: note = l-Biphenylalanine-4-carboxylic acid
  SITE 11: note = (S)-2-amino-3-cyclohexylpropanoic acid
  SITE 13: note = d-2,4-diaminobutyric acid
  SITE 14: note = l-homoTyrosine
XWXGXXDAGXXGXX

SEQ ID NO: 203 - protein, 14 aa, synthetic construct
  SITE 1: note = (S)-2-amino-3-(4-(4-acetylpiperazin-1-yl)phenyl)propanoic acid
  SITE 3: note = l-phenylalanine-4-carboxylic acid
  SITE 5: note = (2S,4R)-4-aminopyrrolidine-2-carboxylic acid
  SITE 6: note = (2S,3S)-2-amino-3-(naphthalen-1-yl)butanoic acid
  SITE 8: note = d-N-methyl-Alanine
  SITE 10: note = l-Biphenylalanine-4-carboxylic acid
  SITE 11: note = l-2,4-diaminobutyric acid
  SITE 13: note = d-Alanine
  SITE 14: note = (S)-2-amino-4-cyclohexylbutanoic acid
XWXGXXDAGXXLAX

SEQ ID NO: 204 - protein, 14 aa, synthetic construct
  SITE 1: note = (S)-2-amino-3-(4-(4-acetylpiperazin-1-yl)phenyl)propanoic acid
  SITE 3: note = l-phenylalanine-4-carboxylic acid
  SITE 5: note = (2S,4R)-4-aminopyrrolidine-2-carboxylic acid
  SITE 6: note = (2S,3S)-2-amino-3-(naphthalen-1-yl)butanoic acid
  SITE 8: note = d-N-methyl-Alanine
  SITE 10: note = l-Biphenylalanine-4-carboxylic acid
  SITE 11: note = (S)-3-acetamido-2-aminopropanoic acid
  SITE 13: note = d-Alanine
  SITE 14: note = (S)-2-amino-4-(5-cyanopyridin-3-yl)butanoic acid
XWXGXXDAGXXKAX

SEQ ID NO: 205 - protein, 14 aa, synthetic construct
  SITE 1: note = (S)-2-amino-3-(4-(4-acetylpiperazin-1-yl)phenyl)propanoic acid
  SITE 3: note = l-phenylalanine-4-carboxylic acid
  SITE 5: note = (2S,4R)-4-aminopyrrolidine-2-carboxylic acid
  SITE 6: note = (2S,3S)-2-amino-3-(naphthalen-1-yl)butanoic acid
  SITE 8: note = d-N-methyl-Alanine
  SITE 10: note = l-Biphenylalanine-4-carboxylic acid
  SITE 11: note = (S)-3-acetamido-2-aminopropanoic acid
  SITE 13: note = d-2,3-diaminopropionic acid
  SITE 14: note = (S)-2-amino-4-(5-cyanopyridin-3-yl)butanoic acid
XWXGXXDAGXXLXX

SEQ ID NO: 206 - protein, 14 aa, synthetic construct
  SITE 1: note = (S)-2-amino-3-(4-(4-acetylpiperazin-1-yl)phenyl)propanoic acid
  SITE 3: note = l-phenylalanine-4-carboxylic acid
  SITE 5: note = (2S,4R)-4-aminopyrrolidine-2-carboxylic acid
  SITE 6: note = (2S,3S)-2-amino-3-(naphthalen-1-yl)butanoic acid
  SITE 8: note = d-N-methyl-Alanine
  SITE 10: note = l-Biphenylalanine-4-carboxylic acid
  SITE 11: note = l-2,3-diaminopropionic acid
  SITE 13: note = d-Alanine
  SITE 14: note = (S)-2-amino-4-cyclohexylbutanoic acid
XWXGXXDAGXXLAX

SEQ ID NO: 207 - protein, 14 aa, synthetic construct
  SITE 1: note = (S)-2-amino-3-(4-(4-acetylpiperazin-1-yl)phenyl)propanoic acid
  SITE 3: note = l-phenylalanine-4-carboxylic acid
  SITE 5: note = (2S,4R)-4-aminopyrrolidine-2-carboxylic acid
  SITE 6: note = (2S,3S)-2-amino-3-(naphthalen-1-yl)butanoic acid
  SITE 8: note = d-N-methyl-Alanine
  SITE 10: note = l-Biphenylalanine-4-carboxylic acid
  SITE 13: note = d-Alanine
  SITE 14: note = (S)-2-amino-4-cyclohexylbutanoic acid
XWXGXXDAGXKLAX

SEQ ID NO: 208 - protein, 14 aa, synthetic construct
  SITE 1: note = (S)-2-amino-3-(4-(4-acetylpiperazin-1-yl)phenyl)propanoic acid
  SITE 3: note = l-phenylalanine-4-carboxylic acid
  SITE 5: note = (2S,4R)-4-aminopyrrolidine-2-carboxylic acid
  SITE 6: note = (2S,3S)-2-amino-3-(naphthalen-1-yl)butanoic acid
  SITE 8: note = d-N-methyl-Alanine
  SITE 10: note = l-Biphenylalanine-4-carboxylic acid
  SITE 11: note = (S)-6-acetamido-2-aminohexanoic acid
  SITE 13: note = d-Alanine
  SITE 14: note = (S)-2-amino-4-(5-cyanopyridin-3-yl)butanoic acid
XWXGXXDAGXKLAX

SEQ ID NO: 209 - protein, 14 aa, synthetic construct
  SITE 1: note = (S)-2-amino-3-(4-(4-acetylpiperazin-1-yl)phenyl)propanoic acid
  SITE 3: note = l-phenylalanine-4-carboxylic acid
  SITE 5: note = (2S,4R)-4-aminopyrrolidine-2-carboxylic acid
  SITE 6: note = (2S,3S)-2-amino-3-(naphthalen-1-yl)butanoic acid
  SITE 8: note = d-N-methyl-Alanine
  SITE 10: note = l-Biphenylalanine-4-carboxylic acid
  SITE 11: note = l-Ornithine
  SITE 13: note = d-Alanine
  SITE 14: note = (S)-2-amino-4-cyclohexylbutanoic acid
XWXGXXDAGXXLAX

SEQ ID NO: 210 - protein, 14 aa, synthetic construct
  SITE 1: note = l-Tyrosine O-ethyl acetamide
  SITE 2: note = (S)-2-amino-3-(6-chloro-1H-indol-3-yl)propanoic acid
  SITE 3: note = l-phenylalanine-4-carboxylic acid
  SITE 5: note = (2S,4R)-4-aminopyrrolidine-2-carboxylic acid
  SITE 6: note = (2S,3S)-2-amino-3-(naphthalen-1-yl)butanoic acid
  SITE 8: note = d-N-methyl-Alanine
  SITE 10: note = l-Biphenylalanine-4-carboxylic acid
  SITE 11: note = (S)-2-amino-3-(1H-pyrrolo[2,3-b]pyridin-3-yl)propanoic acid
  SITE 13: note = d-2,4-diaminobutyric acid
  SITE 14: note = (S)-2-amino-4-cyclohexylbutanoic acid
XXXGXXDAGXXSXX

SEQ ID NO: 211 - protein, 14 aa, synthetic construct
  SITE 1: note = l-Tyrosine O-ethyl acetamide
  SITE 2: note = (S)-2-amino-3-(6-fluoro-1H-indol-3-yl)propanoic acid
  SITE 3: note = l-phenylalanine-4-carboxylic acid
  SITE 5: note = (2S,4R)-4-aminopyrrolidine-2-carboxylic acid
  SITE 6: note = (2S,3S)-2-amino-3-(naphthalen-1-yl)butanoic acid
  SITE 8: note = d-N-methyl-Alanine
  SITE 10: note = l-Biphenylalanine-4-carboxylic acid
  SITE 11: note = (S)-2-amino-3-(indolin-1-yl)propanoic acid
  SITE 13: note = d-2,4-diaminobutyric acid
  SITE 14: note = l-homoTyrosine
XXXGXXDAGXXGXX

SEQ ID NO: 212 - protein, 14 aa, synthetic construct
  SITE 1: note = l-Tyrosine O-ethyl acetamide
  SITE 2: note = (S)-2-amino-3-(6-fluoro-1H-indol-3-yl)propanoic acid
  SITE 3: note = l-phenylalanine-4-carboxylic acid
  SITE 5: note = (2S,4R)-4-aminopyrrolidine-2-carboxylic acid
  SITE 6: note = (2S,3S)-2-amino-3-(naphthalen-1-yl)butanoic acid
  SITE 8: note = d-N-methyl-Alanine
  SITE 10: note = l-Biphenylalanine-4-carboxylic acid
  SITE 11: note = (S)-2-amino-3-(1H-pyrrolo[2,3-b]pyridin-3-yl)propanoic acid
  SITE 13: note = d-2,4-diaminobutyric acid
  SITE 14: note = (S)-2-amino-4-cyclohexylbutanoic acid
XXXGXXDAGXXSXX

SEQ ID NO: 213 - protein, 14 aa, synthetic construct
  SITE 1: note = l-Tyrosine O-ethyl acetamide
  SITE 2: note = (S)-2-amino-3-(6-fluoro-1H-indol-3-yl)propanoic acid
  SITE 3: note = l-phenylalanine-4-carboxylic acid
  SITE 5: note = (2S,4R)-4-aminopyrrolidine-2-carboxylic acid
  SITE 6: note = (2S,3S)-2-amino-3-(naphthalen-1-yl)butanoic acid
  SITE 8: note = d-N-methyl-Alanine
  SITE 10: note = l-Biphenylalanine-4-carboxylic acid
  SITE 11: note = (S)-2-amino-3-(1H-pyrrolo[2,3-b]pyridin-3-yl)propanoic acid
  SITE 13: note = [(R)-3-amino-3-carboxypropyl]-trimethylazanium
  SITE 14: note = (S)-2-amino-4-cyclohexylbutanoic acid
XXXGXXDAGXXSXX

SEQ ID NO: 214 - protein, 14 aa, synthetic construct
  SITE 1: note = l-Tyrosine O-ethyl acetamide
  SITE 3: note = l-phenylalanine-4-carboxylic acid
  SITE 5: note = (2S,4R)-4-aminopyrrolidine-2-carboxylic acid
  SITE 6: note = (2S,3S)-2-amino-3-(naphthalen-1-yl)butanoic acid
  SITE 8: note = d-N-methyl-Alanine
  SITE 10: note = l-Biphenylalanine-4-carboxylic acid
  SITE 11: note = (S)-2-amino-3-(1H-pyrrolo[2,3-b]pyridin-3-yl)propanoic acid
  SITE 13: note = d-2,4-diaminobutyric acid
  SITE 14: note = (S)-2-amino-4-cyclohexylbutanoic acid
XWXGXXDAGXXGXX

SEQ ID NO: 215 - protein, 14 aa, synthetic construct
  SITE 1: note = l-Tyrosine O-ethyl acetamide
  SITE 3: note = l-phenylalanine-4-carboxylic acid
  SITE 5: note = (2S,4R)-4-aminopyrrolidine-2-carboxylic acid
  SITE 6: note = (2S,3S)-2-amino-3-(naphthalen-1-yl)butanoic acid
  SITE 8: note = d-N-methyl-Alanine
  SITE 10: note = l-Biphenylalanine-4-carboxylic acid
  SITE 11: note = (S)-2-amino-3-(1H-pyrrolo[2,3-b]pyridin-3-yl)propanoic acid
  SITE 13: note = d-2,4-diaminobutyric acid
  SITE 14: note = l-homoTyrosine
XWXGXXDAGXXGXX